European Patent Specification EP 4 402 271 B1, published September 10, 2025. Title: TRANSGENIC PLANTS PRODUCING HIGH LEVELS OF APOCAROTENOIDS COMPOUNDS AND USES THEREOF. Applicant: Universidad Castilla La Mancha. Application EP, filed September 15, 2022. The sequence listing filed with the application follows.

SEQUENCE LISTING (38 sequences)

SEQ ID NO: 1 - DNA, 1898 bp, Crocus sativus
  source 1..1898: mol_type = genomic DNA
actattattcttgacatggaatctcctgctactaaattacctgcacctctgctgatgttatcttcttctccattccttctcccttctcctaataagagctcctccatcttccttccacgtaaattagggccgctacctccaaaatattattattacaattgctgccatcctaagagtagatcaatctcagtagtatcaatggcaaataaggaggaggcagagaccagtaagaagaagcccaaaccattaaaagtactaattaccaaagtggatccgaagccgaggaagggcatggcatccgtcgcagtggacttactcgagaaggcctttgtatacctattgtccggaaattctgcagctgatcgtagtagtagtagtggtcgtcgtcgtcgtaaagagcattactacctctccggcaattatgcgcccgtcggacacgaaaccccgccctccgaccacctccccattcatggatcccttcctgaatgcttgaatggagtgtttctgagagttggtcctaaccccaagtttgctcccgtagccggatacaattgggtcgatggagatggaatgattcatggattgcgtattaaagatggaaaagcaacttatctatctcgatatattaaaacgtcacggtttaaacaagaagaatattttggaagagcaaaatttatgaagattggagatctaaggggattgcttgggttctttacgatcttaatactagtacttcgaacaacattgaaagtaatagacatttcatatggaagagggacgggtaatacagctcttgtgtatcataatggcttactattggctctatcagaagaagataaaccttatgttgttaaagttttagaagatggagacttgcaaactcttgggatattggattatgacaagaaattgtcacatccattcaccgctcatccaaagatcgatccgttaactgatgagatgtttacctttggatattccatctcgcctccgtatcttacttatcgagtcatttccaaggatggagtgatgcaagatccagtgcaaatctcaattacatcccctaccataatgcatgattttgctattactgaaaattatgccatcttcatggacctgcccttgtatttccaaccagaggaaatggtaaaggggaaatttgtctcttcatttcaccctacaaaaagagctcgtatcggtgtgcttccacgatatgcaaaagacgagcatccaattcgatggttcgatcttccaagttgcttcatgactcataatgcaaatgcttgggaagagaatgatgaagttgtgctattcacatgtcgccttgagagtcctgatcttgacatgcttagtggacctgcggaagaagagattgggaattcaaaaagtgagctttacgaaatgaggttcaatttgaaaactggaattacttcacaaaagcaactatctgtacctagtgttgattttcctcggatcaaccaaagttatactggcaggaaacagcaatatgtttattgtactcttggcaacaccaagattaagggcattgtgaagtttgatctgcaaattgaaccagaagccggaaagacaatgcttgaagttggaggaaatgtacaaggcatctttgagttgggacctagaagatatggttcagaggcaatatttgtgccatgccaacctggcatcaaatctgatgaggatgacggttacttgatattctttgtacacgacgaaaacaatgggaaatctgaggtcaatgtcatcgatgcaaagacaatgtctgcagaacctgtggctgttgtggaacttccaagcagggttccatatggattccatgccttgtttctgaatgaggaagaacttcagaagcaccaagcagagacatgacaatcactagt

SEQ ID NO: 2 - protein, 623 aa, Crocus sativus
MESPATKLPAPLLMLSSSPFLLPSPNKSSSIFLPRKLGPLPPKYYYYNCCHPKSRSISVVSMANKEEAETSKKKPKPLKVLITKVDPKPRKGMASVAVDLLEKAFVYLLSGNSAADRSSSSGRRRRKEHYYLSGNYAPVGHETPPSDHLPIHGSLPECLNGVFLRVGPNPKFAPVAGYNWVDGDGMIHGLRIKDGKATYLSRYIKTSRFKQEEYFGRAKFMKIGDLRGLLGFFTILILVLRTTLKVIDISYGRGTGNTALVYHNGLLLALSEEDKPYVVKVLEDGDLQTLGILDYDKKLSHPFTAHPKIDPLTDEMFTFGYSISPPYLTYRVISKDGVMQDPVQISITSPTIMHDFAITENYAIFMDLPLYFQPEEMVKGKFVSSFHPTKRARIGVLPRYAKDEHPIRWFDLPSCFMTHNANAWEENDEVVLFTCRLESPDLDMLSGPAEEEIGNSKSELYEMRFNLKTGITSQKQLSVPSVDFPRINQSYTGRKQQYVYCTLGNTKIKGIVKFDLQIEPEAGKTMLEVGGNVQGIFELGPRRYGSEAIFVPCQPGIKSDEDDGYLIFFVHDENNGKSEVNVIDAKTMSAEPVAVVELPSRVPYGFHALFLNEEELQKHQAET

SEQ ID NO: 3 - DNA, 1496 bp, Crocus sativus
  source 1..1496: mol_type = genomic DNA
ggacagccagcagaaatcacaatggacgagaaagatgttgaacggcaacaaatgccacatcctcctcctcccctgtccagcacaaggccatatcaaccccattctccaattcggcaagcgactggcctctcacaacctcctcaccacactcgtcaacacccggttcctctccaactcgaccaaatccgaacccggtccggtcaacatccagtgcatatccgacggattcgatcccggtgggatgaatgcagcacctagtcgtcgggcctatttcgaccgacctcagagtcggtcgggtcagaaacatgttggcctcatcgagtcactccggtccagaggccgacccggcgcatgttttggtctacgacccgttcccctctgggcaatgaacgtagccgagcggtccgggctgcggtcggtcgcattctttactcagccgtgtgcagtggacacaatctaccgccacgtgtgggagggacgaattaaggttccggttgccgagccggtccggttgcctggattgcccccactcgagcctagtgatctgccgtgcgttcgtaacggattcggacgagtcgttaacccggatctcttgccacttcgagtgaatcagcacaaaaatttggacaaagctgacatgatggggaggaactccatatacgagctagaggcggatttgttggatgggtcccgattaccattaccggtgaagtcgattgggccgaccgtgccgtctacttatctcgacaaccgaatcccgtcggattcacactatggattcaatctatacacccctgacactactccctacttggactggctcgactccaaggccccgaactctgtcatctatgtctcatttggtagtttgtccagtctgagccctgatcaaaccaatgagattgcgtcgggtctgatcgccaccaacaaaagctttatttgggtggtacgcacttcggagttagccaaactccctgccaacttcacccaagagaatgcgagccgtgggctggttgtgacctggtgcgaccaactcgatctcctcgcacacgttgcgaccggttgcttcgtgactcactgcggatggaactcgactatggaaggtgtcgcacttggtgtgccgatggtgggagtgccgcagtggtcggaccagcctatgaatgccaagtatgtagaggatgtgtggaaggtcggcgtgagggcgaagacttatgggaaggattttgtgagaggggaggagttcaaaagatgtgtggaggaggtgatggatggagagaggagtggaaagattagagagaatgccgcaaggtggtgtaagttggccaaggactctgttagtgagggtgggagttctgacaagtgtatcaaggagttcatacatcagtgttgcaatgactccaaaatttccttagtttaatcaccctgttaataaagttttgtttcatgtgtcaaacctgagtcaatctattaagagaaaaattgtgcataacagaaga

SEQ ID NO: 4 - protein, 460 aa, Crocus sativus
MLNGNKCHILLLPCPAQGHINPILQFGKRLASHNLLTTLVNTRFLSNSTKSEPGPVNIQCISDGFDPGGMNAAPSRRAYFDRPQSRSGQKHVGLIESLRSRGRPGACFGLRPVPLWAMNVAERSGLRSVAFFTQPCAVDTIYRHVWEGRIKVPVAEPVRLPGLPPLEPSDLPCVRNGFGRVVNPDLLPLRVNQHKNLDKADMMGRNSIYELEADLLDGSRLPLPVKSIGPTVPSTYLDNRIPSDSHYGFNLYTPDTTPYLDWLDSKAPNSVIYVSFGSLSSLSPDQTNEIASGLIATNKSFIWVVRTSELAKLPANFTQENASRGLVVTWCDQLDLLAHVATGCFVTHCGWNSTMEGVALGVPMVGVPQWSDQPMNAKYVEDVWKVGVRAKTYGKDFVRGEEFKRCVEEVMDGERSGKIRENAARWCKLAKDSVSEGGSSDKCIKEFIHQCCNDSKISLV

SEQ ID NO: 5 - DNA, 1548 bp, Crocus sativus
  source 1..1548: mol_type = genomic DNA
atggctgagaaagaagcaaatacccatgtcgtcctcttccccttgccaggccaagggcacatcggctcaatgctgaaactggcacagcttctttccaccgccggattctacgtcactttcgtccacaccgaacgcaactaccgtcgctacctcctcacctccacgtccttccacgtccccaagttccggttccgcaccatccccgacggttttcccgacgacgattcccgctcgcccctcccttttctcgagctccaagagtcgctggacacgaaatgtcgggggcattatcgggaattgttggtcgctgtcgacgaccaagaagagtggcccccagtcacttgtgtcgtggctgatcaagctcttccactctcactcgaagttcccgacgagttggggattcctgtaatgatactcgcaccacacagtgcgtgcagtatattgacgagttattcgattccggagcttataaggggaggtgaactccctatcccagatggggccaatatggatgaactattacaaggcgtactgggattggaaggtatcgtgaggcgtagggatatgtccatcagaagcgccaagtccatccaagatccatttcttcaattcgaagtgaaaatgagcaaaaacttgcccagaggaagagctctcatcctgaacactacagaatcgatagactctctttctttgcgacacattcggtcgatctgtcccactacctacgcactcgggcccttccacgtccttctcaggaacataaaagacgagtcccactccgcaagcctttccgaagaggacaggtcctgcatcgcctggctggactcgaaaccgaacaagtccgcggtctacgtgagtttcggtagcctcgccgccatgccgagagaagcatttcttgagtttcagcagggattgctcgacagcgggtattacttcttgtgggtgatccggcccgatatggtggaaggggggctggaagagagcgagctgaccgcgagcgaacaacgctactttgtgaagtgggccccacaggaggaggttcttgcgcacccggcggtagggtgtttcttgacgcacagcggttggaactctacgttggagagtatctttgcgggagtgccgatgatatgttggcctttctttgcggaccagctgattaacagtaggtttgcgagcgaggtgtggaaaattgccttggatatgaaggatttatgcggaaggagccacgtggagaggatggtgaaggaagttatgagtggagagaaaggcgaagagctaaggaattctagctgcgagatggcagatagggtgaagaagagtgcagaggaaggtggctcttcctatgccaacttcaaagagttggttggacatatcaaatctttgagcttaccagcagaaagaggagaaaatggtggtgaaggaatgagtgtacaagcgccgagtaaacttttcctcctcaacgctgaggacggaaaacatgtccttaaaagtgacgaaccgtcggaacaaaggggtccacaatttaatccaaattttcttcggacctga

SEQ ID NO: 6 - protein, 515 aa, Crocus sativus
MAEKEANTHVVLFPLPGQGHIGSMLKLAQLLSTAGFYVTFVHTERNYRRYLLTSTSFHVPKFRFRTIPDGFPDDDSRSPLPFLELQESLDTKCRGHYRELLVAVDDQEEWPPVTCVVADQALPLSLEVPDELGIPVMILAPHSACSILTSYSIPELIRGGELPIPDGANMDELLQGVLGLEGIVRRRDMSIRSAKSIQDPFLQFEVKMSKNLPRGRALILNTTESIDSLSLRHIRSICPTTYALGPFHVLLRNIKDESHSASLSEEDRSCIAWLDSKPNKSAVYVSFGSLAAMPREAFLEFQQGLLDSGYYFLWVIRPDMVEGGLEESELTASEQRYFVKWAPQEEVLAHPAVGCFLTHSGWNSTLESIFAGVPMICWPFFADQLINSRFASEVWKIALDMKDLCGRSHVERMVKEVMSGEKGEELRNSSCEMADRVKKSAEEGGSSYANFKELVGHIKSLSLPAERGENGGEGMSVQAPSKLFLLNAEDGKHVLKSDEPSEQRGPQFNPNFLRT

SEQ ID NO: 7 - DNA, 2157 bp, synthetic construct
  source 1..2157: mol_type = other DNA; note = pE8 promoter
tccctaatgatattgttcacgtaattaagttttgtggaagtgagagagtccaattttgataagaaaagagtcagaaaacgtaatattttaaaagtctaaatctttctacaaataagagcaaatttatttattttttaatccaataaatattaatggaggacaaattcaattcacttggttgtaaaataaacttaaaccaataaccaaagaactaataaatcctgaagtggaattattaaggataaatgtacatagacaatgaagaaataataggttcgatgaattaataataattaaggatgttacaatcatcatgtgccaagtatatacacaatattctatgggatttataatttcgttacttcacttaacttttgcgtaaataaaacgaattatctgatattttataataaaacagttataagaaccatcatttttaacaacatagatatattatttctaatagtttaatgatacttttaaatcttttaaattttatgtttcttttagaaaataaaaattcaaaaaattaaatatatttacaaaaactacaatcaaacacaacttcatatattaaaagcaaaatatattttgaaaatttcaagtgtcctaacaaataagacaagaggaaaatgtacgatgagagacataaagagaactaataattgaggagtcctataatatataataaagtttattagtaaacttaattattaaggactcctaaaatatatgataggagaaaatgaatggtgagagatattggaaaacttaataattaaggattttaaaatatatggtaaaagataggcaaagtatccattatccccttttaacttgaagtctactaggcgcatgtgaaagttgattttttgtcacgtcatatagctataacgtaaaaaaagaaagtaaaatttttaattttttttaatatatgacatattttaaacgaaatataggacaaaatgtaaatgaatagtaaaggaaacaaagattaatacttactttgtaagaatttaagataaatttaaaatttaatagatcaactttacgtctagaaagacccatatctagaaggaatttcacgaaatcggcccttattcgaaaataacttttaaataatgaattttaaattttaagaaataatatccaatgaataaatgacatgtagcattttacctaaatatttcaactattttaatccaatattaatttgttttattcccaacaatagaaagtcttgtgcagacatttaatctgacttttccagtactaaatattaattttctgaagattttcgggtttagtccacaagttttagtgagaagttttgctcaaattttaggtgagaaggtttgatatttatcttttgttaaattaatttatctaggtgactattatttatttaagtagaaattcatatcattacttttgccaacttgtagtcataataggagtaggtgtatatgatgaaggaataaacaagttcagtgaagtgattaaaataaaatataatttaggtgtacatcaaataaaaaccttaaagtttagaaaggcaccgaataattttgcatagaagatattagtaaatttataaaaataaaagaaatgtagttgtcaagttgtcttcttttttttggataaaaatagcagttggcttatgtcattcttttacaacctccatgccacttgtccaattgttgacacttaactaattagtttgattcatgtatgaatactaaataattttttaggactgactcaaatatttttatattatcatagtaatatttatctaatttttaggaccacttattactaaataataaattaactacaactatattattgttgtgaaacaacaacgttttggttgttatgatgaaacgtacactatatcagtatgaaaaattcaaaacgattagtataaattatattgaaaatttgatatttttctattcttaatcagacgtattgggtttcatattttaaaaagggactaaacttagaagagaagtttgtttgaaactacttttgtctctttcttgttcccatttctctcttagatttcaaaaagtgaactactttatctccttctttgttcacattttattttattctattataaatatggcatcctcatattgagatttttag

SEQ ID NO: 8 - DNA, 4034 bp, synthetic construct
  source 1..4034: mol_type = other DNA; note = p2A11 promoter
gtcaaacaattttgaggaattcaatttcatctttaactggtacaataatcattttatcatgaaaataagcagctcaagagaatttttgaagaatcttttatttctttaacatttaaccacatgaatttttaatttttttttgcaatacatttaaaccgaaatggtcaaacgatcaaccaactgatctttattctaataaacttctagtttacatttgcatgtgagtgcatcatcattatcatatttgtacacaacaaacaagaaaaaaatataaacaatattttatttaaatatttatattccactttgactgtagatattaaatcttgtcatcatttatagtctcaatattataatttttttattttttcaaaattcaaaagtttacaattatttttttgaactataatattatccaagatgaacatctcaagaagaaaattattaatattgttatggttaaaattttacatacaatacttgttttttgctttacttttatcttaccgtagatacacaatcgacgataacttagtgatcacacaataataattattttgttcatgacacaatatttataagaaatacttatttctttcttttatccttcagtagttcataataaaaacataccataatatttgtgatgcattcatagtacgtaatgaaatgacaatttatgtcaaattattttcttttatactctcaaacctcccgtaaaggtgagatgagtcatttatccaattatacataaatatgtctttattcatgctctttatcacattctgacacattcacttaatttcaagagtaagcaagcatgataactgaaactatttatgcgtatcttaccttgatatttgacacattacatgacacacctcaacatcactttcaaagattaagcgcaccaccatattatctttctttttttttttatgaaggttttataaaattattaaattaggtccaaaaaattgtttgtcaaataaccttttatactagattgatgacaaaaattacctttacgttttgaaagaccattttaagacctaatctatcagtgactccttaaagttggcacaatatttcacttagacaccctaattgaatgatgttcattttaaacacccaatgtagggttccgctatatcattttgacacatttcttaacatcaacaaaaatatataatgagtatgtgatatactcgcgaatgacgtgaaaaatgaagacatttgttatttgtatcaaagtagttactaaataattaattttgaataaaaataaaagctgaccagtaaatcaataacacataatattttccacctaataattaaaatataaaataaaaaagagccatctcagggtcatctgcccaccattgctatttcaaagaaatttgtacgttagtttatagaaattgatgttaaaattctttcaagaaaaatttatgaatgaatttattctctaatttaaaaatattttctgttatttttgttgaaagaaatttaacttggataaaatggtggttaaaactggaaagaagaaaagagaaaaaataattaaaaatcatttcacgctctaatcaatgagcgtatcacattcattatgttatataagcaaaagtgacaaaacgaaaataatatattacatgaaatgtctaaaataaatatcgtctaattaaaatatctaagtaacatattgtgcctaactttagagggatcatcaataagttaaaccccattttaataactcataattgtcctttttatttaatattgtcacaaatcacaatgataattaacattaatttgtcctttgtgacgtccatattcatgcatttaaccaatcatcttcatttggacttattatcacaattatcccactttcctcacaaaatggagcattcaagtggaatagactacacgatttttaatttcatcaaaaacatctttttgctttattcattattatattgtcgctattgttgaattttatttgccctaaatttcttaccataaatagatttttcttttagaaaaaggagattgactaattcttttcttgtaggaaaaggtttaggactctataaatagagacatattccttctaacttaatcaacatttacaatgtagtcttaaagactttgaaagtttttggttagggggagaaattgtgggtcacaagcttgatacgttatcaattgtgtaaacctcccatgtattctgagtgaatttggttgaggttgtttccctctgtattttgtactctcatatttatagtggattgttcatctctttcgtggacgtaggtcgattgaccgtcgattgaccgaaccacgttaaatctttgtattttttgatatatttctcattatcttcttactcgtgatctttcaaggtttgcattgctatcttccgcgttacaccaacttatttacgatcctaacagctatggtgtggaaacataaatcaaacattttactgatataaacacatctttgattataacatgatagaaatttgagcccaactttttatcatcattatatacaaaaagttctaaattttttttttgatgtagtaaaacttaaatccatagtcttgcccctaaaccaatgacataatatataacccaaaatatactagttttcgccctcgagccctttaaaaagtatagtcaatatttacggtgaccgtgaatttcttaattatgatatataatttaaaagaaatcatgatcacattctactgatgagaacatgtgctaatcaagggaaaacatggatgtgaaaaatactttttgttaaaagtaaaaaaaaatgtgaaattttgttagttatttactacctatacattatttgagcatgtgcaaactttacaaatacctaatagaagattttcacctgcctgtatatatgtaaattaattataatgaacactctcacataaaataattatcagtatatacattaatacttgccctccacaatgaattaaataaaatgtagaacatgatctacacttcaataaaactaagaccataaagaataatttcaaaatatacacatgtcaacaataaattatttgcatattatattaacttactaaacaatctttacttttgaaatataaaaataatcaagttataagtctgctcaaagtaaagcacttgttagactcatctgattttgagaaggtaagcaaattgatggtgcataatagtcacaagtaaaatataaaatagatttcattagtaaaattgttttttactttctttatatataattatcaatatccttcaatggtaggttaattatattgttaacttcttgttgaattaaagcaataagacaagaatattaaagataaaagaacaataaaaatagaaagactaagagataagagttttcttattcttctttcaataagtatcatcaagtgtatacaatataaatttttgtatttttgatctatctatttataatgttatatataagcatacaaaagatcagtcataaatatgactttaatcatgaaaataatgaaagagattatgaaggcgtaaggttactagaataatagtcattaaaaaaaggggttatctttataattgaataattgatgaagtaatggagataattagtgagcataaatttttttaaaaaaatggacatttacactataatattttataacactttcccttaaacatctaggtataaataatgagtcttgtcaaaatcttagtaggaaaaattctgtgaaatttttttagtgaaaacaaatgatataaatatcttgaatactcattatttgttgtctcattaaaaatcttatctgacctataaaataaattatttgctcaactcaaaatagtttttcattctaaaattagtataattattagtgaatatttaattaacataattgtatactaaggggcctataaattggattcttctcaaagaaaaataaaatcaccacacaactttcttcttctgctcatcaattagcaattaatccaaaacca

SEQ ID NO: 9 - DNA, 1027 bp, synthetic construct
  source 1..1027: mol_type = other DNA; note = p35S promoter
actagagccaagctgatctcctttgccccggagatcaccatggacgactttctctatctctacgatctaggaagaaagttcgacggagaaggtgacgataccatgttcaccaccgataatgagaagattagcctcttcaatttcagaaagaatgctgacccacagatggttagagaggcctacgcggcaggtctgatcaagacgatctacccgagtaataatctccaggagatcaaataccttcccaagaaggttaaagatgcagtcaaaagattcaggactaactgcatcaagaacacagagaaagatatatttctcaagatcagaagtactattccagtatggacgattcaaggcttgcttcataaaccaaggcaagtaatagagattggagtctctaagaaagtagttcctactgaatcaaaggccatggagtcaaaaattcagatcgaggatctaacagaactcgccgtgaagactggcgaacagttcatacagagtcttttacgactcaatgacaagaagaaaatcttcgtcaacatggtggagcacgacactctcgtctactccaagaatatcaaagatacagtctcagaagaccaaagggctattgagacttttcaacaaagggtaatatcgggaaacctcctcggattccattgcccagctatctgtcacttcatcaaaaggacagtagaaaaggaaggtggcacctacaaatgccatcattgcgataaaggaaaggctatcgttcaagatgcctctgccgacagtggtcccaaagatggacccccacccacgaggagcatcgtggaaaaagaagacgttccaaccacgtcttcaaagcaagtggattgatgtgatatctccactgacgtaagggatgacgcacaatcccactatccttcgcaagacccttcctctatataaggaagttcatttcatttggagaggactccggtatttttacaacaataccacaacaaaacaaacaacaaacaacattacaatttactattctagtcga

SEQ ID NO: 10 - DNA, 37 bp, synthetic construct
  source 1..37: mol_type = other DNA; note = forward primer pUPD2-Dom-UGT2-F
gcgccgtctcgctcgaatgttgaacggcaacaaatgc

SEQ ID NO: 11 - DNA, 45 bp, synthetic construct
  source 1..45: mol_type = other DNA; note = Reverse pPrimer pUPD2-Dom-UGT2-R
gcgccgtctcgctcaaagcttaaactaaggaaattttggagtcat

SEQ ID NO: 12 - DNA, 40 bp, synthetic construct
  source 1..40: mol_type = other DNA; note = Forward primer pUPD2-Dom-CsCCD2-L-F1
gcgccgtctcgctcgaatggaatctcctgctactaaatta

SEQ ID NO: 13 - DNA, 31 bp, synthetic construct
  source 1..31: mol_type = other DNA; note = Reverse primer pUPD2-Dom-CsCCD2-L-R1
gcgccgtctcgttgtctctgcctcctcctta

SEQ ID NO: 14 - DNA, 33 bp, synthetic construct
  source 1..33: mol_type = other DNA; note = Forward primer pUPD2-Dom-CsCCD2-L-F2
gcgccgtctcgacaagtaagaagaagcccaaac

SEQ ID NO: 15 - DNA, 39 bp, synthetic construct
  source 1..39: mol_type = other DNA; note = Reverse primer pUPD2-Dom-CsCCD2-L-R2
gcgccgtctcgctcaaagctcatgtctctgcttggtgct

SEQ ID NO: 16 - DNA, 39 bp, synthetic construct
  source 1..39: mol_type = other DNA; note = Forward primer pUPD2-Dom-UGT709-F
gcgccgtctcgctcgaatggctgagaaagaagcaaatac

SEQ ID NO: 17 - DNA, 40 bp, synthetic construct
  source 1..40: mol_type = other DNA; note = Reverse primer pUPD2-Dom-UGT709-R
gcgccgtctcgctcaaagctcaggtccgaagaaaatttgg

SEQ ID NO: 18 - DNA, 3978 bp, synthetic construct
  source 1..3978: mol_type = other DNA; plasmid = pUPD2-CsCCD2L
aatggaatctcctgctactaaattacctgcacctctgctgatgttatcttcttctccattccttctcccttctcctaataagagctcctccatcttccttccacgtaaattagggccgctacctccaaaatattattattacaattgctgccatcctaagagtagatcaatctcagtagtatcaatggcaaataaggaggaggcagagacaagtaagaagaagcccaaaccattaaaagtactaattaccaaagtggatccgaagccgaggaagggcatggcatccgtcgcagtggacttactcgagaaggcctttgtatacctattgtccggaaattctgcagctgatcgtagtagtagtagtggtcgtcgtcgtcgtaaagagcattactacctctccggcaattatgcgcccgtcggacacgaaaccccgccctccgaccacctccccattcatggatcccttcctgaatgcttgaatggagtgtttctgagagttggtcctaaccccaagtttgctcccgtagccggatacaattgggtcgatggagatggaatgattcatggattgcgtattaaagatggaaaagcaacttatctatctcgatatattaaaacgtcacggtttaaacaagaagaatattttggaagagcaaaatttatgaagattggagatctaaggggattgcttgggttctttacgatcttaatactagtacttcgaacaacattgaaagtaatagacatttcatatggaagagggacgggtaatacagctcttgtgtatcataatggcttactattggctctatcagaagaagataaaccttatgttgttaaagttttagaagatggagacttgcaaactcttgggatattggattatgacaagaaattgtcacatccattcaccgctcatccaaagatcgatccgttaactgatgagatgtttacctttggatattccatctcgcctccgtatcttacttatcgagtcatttccaaggatggagtgatgcaagatccagtgcaaatctcaattacatcccctaccataatgcatgattttgctattactgaaaattatgccatcttcatggacctgcccttgtatttccaaccagaggaaatggtaaaggggaaatttgtctcttcatttcaccctacaaaaagagctcgtatcggtgtgcttccacgatatgcaaaagacgagcatccaattcgatggttcgatcttccaagttgcttcatgactcataatgcaaatgcttgggaagagaatgatgaagttgtgctattcacatgtcgccttgagagtcctgatcttgacatgcttagtggacctgcggaagaagagattgggaattcaaaaagtgagctttacgaaatgaggttcaatttgaaaactggaattacttcacaaaagcaactatctgtacctagtgttgattttcctcggatcaaccaaagttatactggcaggaaacagcaatatgtttattgtactcttggcaacaccaagattaagggcattgtgaagtttgatctgcaaattgaaccagaagccggaaagacaatgcttgaagttggaggaaatgtacaaggcatctttgagttgggacctagaagatatggttcagaggcaatatttgtgccatgccaacctggcatcaaatctgatgaggatgacggttacttgatattctttgtacacgacgaaaacaatgggaaatctgaggtcaatgtcatcgatgcaaagacaatgtctgcagaacctgtggctgttgtggaacttccaagcagggttccatatggattccatgccttgtttctgaatgaggaagaacttcagaagcaccaagcagagacatgagctttgagaccactcatcgcgactagtagcggccgctgcagtccggcaaaaaagggcaaggtgtcaccaccctgccctttttctttaaaaccgaaaagattacttcgcgttatgcaggcttcctcgctcactgactcgctgcgctcggtcgttcggctgcggcgagcggtatcagctcactcaaaggcggtaatacggttatccacagaatcaggggataacgcaggaaagaacatgtgagcaaaaggccagcaaaaggccaggaaccgtaaaaaggccgcgttgctggcgtttttccacaggctccgcccccctgacgagcatcacaaaaatcgacgctcaagtcagaggtggcgaaacccgacaggactataaagataccaggcgtttccccctggaagctccctcgtgcgctctcctgttccgaccctgccgcttaccggatacctgtccgcctttctcccttcgggaagcgtggcgctttctcatagctcacgctgtaggtatctcagttcggtgtaggtcgttcgctccaagctgggctgtgtgcacgaaccccccgttcagcccgaccgctgcgccttatccggtaactatcgtcttgagtccaacccggtaagacacgacttatcgccactggcagcagccactggtaacaggattagcagagcgaggtatgtaggcggtgctacagagttcttgaagtggtggcctaactacggctacactagaagaacagtatttggtatctgcgctctgctgaagccagttaccttcggaaaaagagttggtagctcttgatccggcaaacaaaccaccgctggtagcggtggtttttttgtttgcaagcagcagattacgcgcagaaaaaaaggatctcaagaagatcctttgatcttttctacggggtctgacgctcagtggaacgaaaactcacgttaagggattttggtcatgagattatcaaaaaggatcttcacctagatccttttaaattaaaaatgaagttttaaatcaatctaaagtatatatgagtaaacttggtctgacagctcgaggcttggattctcaccaataaaaaacgcccggcggcaaccgagcgttctgaacaaatccagatggagttctgaggtcattactggatctatcaacaggagtccaagcgagctcgatatcaaattacgccccgccctgccactcgtcgcagtactgttgtaattcattaagcattctgccgacatggaagccatcacaaacggcatgatgaacctgaatcgccagcggcatcagcaccttgtcgccttgcgtataatatttgcccatggtgaaaacgggggcgaagaagttgtccatattggccacgtttaaatcaaaactggtgaaactcacccagggattggctgatacgaaaaacatattctcaataaaccctttagggaaataggccaggttttcaccgtaacacgccacatcttgcgaatatatgtgtagaaactgccggaaatcgtcgtggtattcactccagagtgatgaaaacgtttcagtttgctcatggaaaacggtgtaacaagggtgaacactatcccatatcaccagctcaccgtctttcattgccatacgaaattccggatgagcattcatcaggcgggcaagaatgtgaataaaggccggataaaacttgtgcttatttttctttacggtctttaaaaaggccgtaatatccagctgaacggtctggttataggtacattgagcaactgactgaaatgcctcaaaatgttctttacgatgccattgggatatatcaacggtggtatatccagtgatttttttctccattttagcttccttagctcctgaaaatctcgataactcaaaaaatacgcccggtagtgatcttatttcattatggtgaaagttggaacctcttacgtgcccgatcaactcgagtgccacctgacgtctaagaaaccattattatcatgacattaacctataaaaataggcgtatcacgaggcagaatttcagataaaaaaaatccttagctttcgctaaggatgatttctggaattcgcggccgcttctagagcgatgagtggtctcg

SEQ ID NO: 19 - DNA, 3489 bp, synthetic construct
  source 1..3489: mol_type = other DNA; plasmid = pUPD2-CsUGT2
aatgttgaacggcaacaaatgccacatcctcctcctcccctgtccagcacaaggccatatcaaccccattctccaattcggcaagcgactggcctctcacaacctcctcaccacactcgtcaacacccggttcctctccaactcgaccaaatccgaacccggtccggtcaacatccagtgcatatccgacggattcgatcccggtgggatgaatgcagcacctagtcgtcgggcctatttcgaccgacctcagagtcggtcgggtcagaaacatgttggcctcatcgagtcactccggtccagaggccgacccggcgcatgttttggtctacgacccgttcccctctgggcaatgaacgtagccgagcggtccgggctgcggtcggtcgcattctttactcagccgtgtgcagtggacacaatctaccgccacgtgtgggagggacgaattaaggttccggttgccgagccggtccggttgcctggattgcccccactcgagcctagtgatctgccgtgcgttcgtaacggattcggacgagtcgttaacccggatctcttgccacttcgagtgaatcagcacaaaaatttggacaaagctgacatgatggggaggaactccatatacgagctagaggcggatttgttggatgggtcccgattaccattaccggtgaagtcgattgggccgaccgtgccgtctacttatctcgacaaccgaatcccgtcggattcacactatggattcaatctatacacccctgacactactccctacttggactggctcgactccaaggccccgaactctgtcatctatgtctcatttggtagtttgtccagtctgagccctgatcaaaccaatgagattgcgtcgggtctgatcgccaccaacaaaagctttatttgggtggtacgcacttcggagttagccaaactccctgccaacttcacccaagagaatgcgagccgtgggctggttgtgacctggtgcgaccaactcgatctcctcgcacacgttgcgaccggttgcttcgtgactcactgcggatggaactcgactatggaaggtgtcgcacttggtgtgccgatggtgggagtgccgcagtggtcggaccagcctatgaatgccaagtatgtagaggatgtgtggaaggtcggcgtgagggcgaagacttatgggaaggattttgtgagaggggaggagttcaaaagatgtgtggaggaggtgatggatggagagaggagtggaaagattagagagaatgccgcaaggtggtgtaagttggccaaggactctgttagtgagggtgggagttctgacaagtgtatcaaggagttcatacatcagtgttgcaatgactccaaaatttccttagtttaagctttgagaccactcatcgcgactagtagcggccgctgcagtccggcaaaaaagggcaaggtgtcaccaccctgccctttttctttaaaaccgaaaagattacttcgcgttatgcaggcttcctcgctcactgactcgctgcgctcggtcgttcggctgcggcgagcggtatcagctcactcaaaggcggtaatacggttatccacagaatcaggggataacgcaggaaagaacatgtgagcaaaaggccagcaaaaggccaggaaccgtaaaaaggccgcgttgctggcgtttttccacaggctccgcccccctgacgagcatcacaaaaatcgacgctcaagtcagaggtggcgaaacccgacaggactataaagataccaggcgtttccccctggaagctccctcgtgcgctctcctgttccgaccctgccgcttaccggatacctgtccgcctttctcccttcgggaagcgtggcgctttctcatagctcacgctgtaggtatctcagttcggtgtaggtcgttcgctccaagctgggctgtgtgcacgaaccccccgttcagcccgaccgctgcgccttatccggtaactatcgtcttgagtccaacccggtaagacacgacttatcgccactggcagcagccactggtaacaggattagcagagcgaggtatgtaggcggtgctacagagttcttgaagtggtggcctaactacggctacactagaagaacagtatttggtatctgcgctctgctgaagccagttaccttcggaaaaagagttggtagctcttgatccggcaaacaaaccaccgctggtagcggtggtttttttgtttgcaagcagcagattacgcgcagaaaaaaaggatctcaagaagatcctttgatcttttctacggggtctgacgctcagtggaacgaaaactcacgttaagggattttggtcatgagattatcaaaaaggatcttcacctagatccttttaaattaaaaatgaagttttaaatcaatctaaagtatatatgagtaaacttggtctgacagctcgaggcttggattctcaccaataaaaaacgcccggcggcaaccgagcgttctgaacaaatccagatggagttctgaggtcattactggatctatcaacaggagtccaagcgagctcgatatcaaattacgccccgccctgccactcgtcgcagtactgttgtaattcattaagcattctgccgacatggaagccatcacaaacggcatgatgaacctgaatcgccagcggcatcagcaccttgtcgccttgcgtataatatttgcccatggtgaaaacgggggcgaagaagttgtccatattggccacgtttaaatcaaaactggtgaaactcacccagggattggctgatacgaaaaacatattctcaataaaccctttagggaaataggccaggttttcaccgtaacacgccacatcttgcgaatatatgtgtagaaactgccggaaatcgtcgtggtattcactccagagtgatgaaaacgtttcagtttgctcatggaaaacggtgtaacaagggtgaacactatcccatatcaccagctcaccgtctttcattgccatacgaaattccggatgagcattcatcaggcgggcaagaatgtgaataaaggccggataaaacttgtgcttatttttctttacggtctttaaaaaggccgtaatatccagctgaacggtctggttataggtacattgagcaactgactgaaatgcctcaaaatgttctttacgatgccattgggatatatcaacggtggtatatccagtgatttttttctccattttagcttccttagctcctgaaaatctcgataactcaaaaaatacgcccggtagtgatcttatttcattatggtgaaagttggaacctcttacgtgcccgatcaactcgagtgccacctgacgtctaagaaaccattattatcatgacattaacctataaaaataggcgtatcacgaggcagaatttcagataaaaaaaatccttagctttcgctaaggatgatttctggaattcgcggccgcttctagagcgatgagtggtctcg

SEQ ID NO: 20 - DNA, 3654 bp, synthetic construct
  source 1..3654: mol_type = other DNA; plasmid = pUPD2-UGT709
aatggctgagaaagaagcaaatacccatgtcgtcctcttccccttgccaggccaagggcacatcggctcaatgttgaaactggcacagcttctttccaccgccggattctacgtcactttcgtccacaccgaacgcaactaccgtcgctacctcctcacctccacgtccttccacgtccccaagttccggttccgcaccatccccgacggttttcccgacgacgattcccgctcgcccctcccttttctcgagctccaagagtcgctggacacgaaatgtcgggggcattatcgggaattgttggtcgctgtcgacgaccaagaagagtggcccccagtcacttgtgtcgtggctgatcaagctcttccactctcactcgaagttcccgacgagttggggattcctgtaatgatactcgcaccacacagtgcgtgcagtatattgacgagttattcgattccggagcttataaggggaggtgaactccctatcccagatggggccaatatggatgaactattacaaggcgtactgggattggaaggtatcgtgaggcgtagggatatgtccatcagaagcgccaagtccatccaagatccatttcttcaattcgaagtgaaaatgagcaaaaacttgcccagaggaagagctctcatcctgaacactacagaatcgatagactctctttctttgcgacacattcggtcgatctgtcccactacctacgcactcgggcccttccacgtccttctcaggaacataaaagacgagtcccactccgcaagcctttccgaagaggacaggtcctgcatcgcctggctggactcgaaaccgaacaagtccgcggtctacgtgagtttcggtagcctcgccgccatggcgagagaagcatttcttgagtttcagcagggattgctcgacagcgggtattacttcttgtgggtgatccggcccgatatggtggaaggggggctggaagagagcgagctgaccgcgagcgaacaacgctactttgtgaagtgggccccacaggaggaggttcttgcgcacccggcggtagggtgtttcttgacgcacagcggttggaactctacgttggagagtatctttgcgggagtgccgatgatatgttggcctttctttgcggaccagctgattaacagtaggtttgcgagcgaggtgtggaaaattgccttggatatgaaggatttgtgcggaaggagccacgtggagaggatggtgaaggaagttatgagtggagagaaaggcgaagagctaaggaattctagctgcgagatggcagatagggtgaagaagagtgcagaggaaggtggctcttcctacgccaacttcaaagagttggttggacatatcaaatctttgagcttaccagcagaaagaggagaaaatggtggtgaaggaatgagtgtacaagcgccgagtaaacttttcctcctcaacgctgaggacggaaaacatgtccttaaaagtgacgaaccgtcggaacaaaggggtccacaatttaatccaaattttcttcggacctgagctttgagaccactcatcgcgactagtagcggccgctgcagtccggcaaaaaagggcaaggtgtcaccaccctgccctttttctttaaaaccgaaaagattacttcgcgttatgcaggcttcctcgctcactgactcgctgcgctcggtcgttcggctgcggcgagcggtatcagctcactcaaaggcggtaatacggttatccacagaatcaggggataacgcaggaaagaacatgtgagcaaaaggccagcaaaaggccaggaaccgtaaaaaggccgcgttgctggcgtttttccacaggctccgcccccctgacgagcatcacaaaaatcgacgctcaagtcagaggtggcgaaacccgacaggactataaagataccaggcgtttccccctggaagctccctcgtgcgctctcctgttccgaccctgccgcttaccggatacctgtccgcctttctcccttcgggaagcgtggcgctttctcatagctcacgctgtaggtatctcagttcggtgtaggtcgttcgctccaagctgggctgtgtgcacgaaccccccgttcagcccgaccgctgcgccttatccggtaactatcgtcttgagtccaacccggtaagacacgacttatcgccactggcagcagccactggtaacaggattagcagagcgaggtatgtaggcggtgctacagagttcttgaagtggtggcctaactacggctacactagaagaacagtatttggtatctgcgctctgctgaagccagttaccttcggaaaaagagttggtagctcttgatccggcaaacaaaccaccgctggtagcggtggtttttttgtttgcaagcagcagattacgcgcagaaaaaaaggatctcaagaagatcctttgatcttttctacggggtctgacgctcagtggaacgaaaactcacgttaagggattttggtcatgagattatcaaaaaggatcttcacctagatccttttaaattaaaaatgaagttttaaatcaatctaaagtatatatgagtaaacttggtctgacagctcgaggcttggattctcaccaataaaaaacgcccggcggcaaccgagcgttctgaacaaatccagatggagttctgaggtcattactggatctatcaacaggagtccaagcgagctcgatatcaaattacgccccgccctgccactcgtcgcagtactgttgtaattcattaagcattctgccgacatggaagccatcacaaacggcatgatgaacctgaatcgccagcggcatcagcaccttgtcgccttgcgtataatatttgcccatggtgaaaacgggggcgaagaagttgtccatattggccacgtttaaatcaaaactggtgaaactcacccagggattggctgatacgaaaaacatattctcaataaaccctttagggaaataggccaggttttcaccgtaacacgccacatcttgcgaatatatgtgtagaaactgccggaaatcgtcgtggtattcactccagagtgatgaaaacgtttcagtttgctcatggaaaacggtgtaacaagggtgaacactatcccatatcaccagctcaccgtctttcattgccatacgaaattccggatgagcattcatcaggcgggcaagaatgtgaataaaggccggataaaacttgtgcttatttttctttacggtctttaaaaaggccgtaatatccagctgaacggtctggttataggtacattgagcaactgactgaaatgcctcaaaatgttctttacgatgccattgggatatatcaacggtggtatatccagtgatttttttctccattttagcttccttagctcctgaaaatctcgataactcaaaaaatacgcccggtagtgatcttatttcattatggtgaaagttggaacctcttacgtgcccgatcaactcgagtgccacctgacgtctaagaaaccattattatcatgacattaacctataaaaataggcgtatcacgaggcagaatttcagataaaaaaaatccttagctttcgctaaggatgatttctggaattcgcggccgcttctagagcgatgagtggtctcg

SEQ ID NO: 21 - DNA, 17969 bp, synthetic construct
  source 1..17969: mol_type = other DNA; plasmid = DNA construct O1= pDGB3alpha1[p35S:UGT2:T35S-p35S:UGT709G1:T35S-pE8:CCD2L:T35S-pNos:Hyg:T35S]
ggagactagagccaagctgatctcctttgccccggagatcaccatggacgactttctctatctctacgatctaggaagaaagttcgacggagaaggtgacgataccatgttcaccaccgataatgagaagattagcctcttcaatttcagaaagaatgctgacccacagatggttagagaggcctacgcggcaggtctgatcaagacgatctacccgagtaataatctccaggagatcaaataccttcccaagaaggttaaagatgcagtcaaaagattcaggactaactgcatcaagaacacagagaaagatatatttctcaagatcagaagtactattccagtatggacgattcaaggcttgcttcataaaccaaggcaagtaatagagattggagtctctaagaaagtagttcctactgaatcaaaggccatggagtcaaaaattcagatcgaggatctaacagaactcgccgtgaagactggcgaacagttcatacagagtcttttacgactcaatgacaagaagaaaatcttcgtcaacatggtggagcacgacactctcgtctactccaagaatatcaaagatacagtctcagaagaccaaagggctattgagacttttcaacaaagggtaatatcgggaaacctcctcggattccattgcccagctatctgtcacttcatcaaaaggacagtagaaaaggaaggtggcacctacaaatgccatcattgcgataaaggaaaggctatcgttcaagatgcctctgccgacagtggtcccaaagatggacccccacccacgaggagcatcgtggaaaaagaagacgttccaaccacgtcttcaaagcaagtggattgatgtgatatctccactgacgtaagggatgacgcacaatcccactatccttcgcaagacccttcctctatataaggaagttcatttcatttggagaggactccggtatttttacaacaataccacaacaaaacaaacaacaaacaacattacaatttactattctagtcgaaatgttgaacggcaacaaatgccacatcctcctcctcccctgtccagcacaaggccatatcaaccccattctccaattcggcaagcgactggcctctcacaacctcctcaccacactcgtcaacacccggttcctctccaactcgaccaaatccgaacccggtccggtcaacatccagtgcatatccgacggattcgatcccggtgggatgaatgcagcacctagtcgtcgggcctatttcgaccgacctcagagtcggtcgggtcagaaacatgttggcctcatcgagtcactccggtccagaggccgacccggcgcatgttttggtctacgacccgttcccctctgggcaatgaacgtagccgagcggtccgggctgcggtcggtcgcattctttactcagccgtgtgcagtggacacaatctaccgccacgtgtgggagggacgaattaaggttccggttgccgagccggtccggttgcctggattgcccccactcgagcctagtgatctgccgtgcgttcgtaacggattcggacgagtcgttaacccggatctcttgccacttcgagtgaatcagcacaaaaatttggacaaagctgacatgatggggaggaactccatatacgagctagaggcggatttgttggatgggtcccgattaccattaccggtgaagtcgattgggccgaccgtgccgtctacttatctcgacaaccgaatcccgtcggattcacactatggattcaatctatacacccctgacactactccctacttggactggctcgactccaaggccccgaactctgtcatctatgtctcatttggtagtttgtccagtctgagccctgatcaaaccaatgagattgcgtcgggtctgatcgccaccaacaaaagctttatttgggtggtacgcacttcggagttagccaaactccctgccaacttcacccaagagaatgcgagccgtgggctggttgtgacctggtgcgaccaactcgatctcctcgcacacgttgcgaccggttgcttcgtgactcactgcggatggaactcgactatggaaggtgtcgcacttggtgtgccgatggtgggagtgccgcagtggtcggaccagcctatgaatgccaagtatgtagaggatgtgtggaaggtcggcgtgagggcgaagacttatgggaaggattttgtgagaggggaggagttcaaaagatgtgtggaggaggtgatggatggagagaggagtggaaagattagagagaatgccgcaaggtggtgtaagttggccaaggactctgttagtgagggtgggagttctgacaagtgtatcaaggagttcatacatcagtgttgcaatgactccaaaatttccttagtttaagcttcggccatgctagagtccgcaaaaatcaccagtctctctctacaaatctatctctctctatttttctccagaataatgtgtgagtagttcccagataagggaattagggttcttatagggtttcgctcatgtgttgagcatataagaaacccttagtatgtatttgtatttgtaaaatacttctatcaataaaatttctaattcctaaaaccaaaatccagtgacctcgctgtcaggagactagagccaagctgatctcctttgccccggagatcaccatggacgactttctctatctctacgatctaggaagaaagttcgacggagaaggtgacgataccatgttcaccaccgataatgagaagattagcctcttcaatttcagaaagaatgctgacccacagatggttagagaggcctacgcggcaggtctgatcaagacgatctacccgagtaataatctccaggagatcaaataccttcccaagaaggttaaagatgcagtcaaaagattcaggactaactgcatcaagaacacagagaaagatatatttctcaagatcagaagtactattccagtatggacgattcaaggcttgcttcataaaccaaggcaagtaatagagattggagtctctaagaaagtagttcctactgaatcaaaggccatggagtcaaaaattcagatcgaggatctaacagaactcgccgtgaagactggcgaacagttcatacagagtcttttacgactcaatgacaagaagaaaatcttcgtcaacatggtggagcacgacactctcgtctactccaagaatatcaaagatacagtctcagaagaccaaagggctattgagacttttcaacaaagggtaatatcgggaaacctcctcggattccattgcccagctatctgtcacttcatcaaaaggacagtagaaaaggaaggtggcacctacaaatgccatcattgcgataaaggaaaggctatcgttcaagatgcctctgccgacagtggtcccaaagatggacccccacccacgaggagcatcgtggaaaaagaagacgttccaaccacgtcttcaaagcaagtggattgatgtgatatctccactgacgtaagggatgacgcacaatcccactatccttcgcaagacccttcctctatataaggaagttcatttcatttggagaggactccggtatttttacaacaataccacaacaaaacaaacaacaaacaacattacaatttactattctagtcgaaatggctgagaaagaagcaaatacccatgtcgtcctcttccccttgccaggccaagggcacatcggctcaatgttgaaactggcacagcttctttccaccgccggattctacgtcactttcgtccacaccgaacgcaactaccgtcgctacctcctcacctccacgtccttccacgtccccaagttccggttccgcaccatccccgacggttttcccgacgacgattcccgctcgcccctcccttttctcgagctccaagagtcgctggacacgaaatgtcgggggcattatcgggaattgttggtcgctgtcgacgaccaagaagagtggcccccagtcacttgtgtcgtggctgatcaagctcttccactctcactcgaagttcccgacgagttggggattcctgtaatgatactcgcaccacacagtgcgtgcagtatattgacgagttattcgattccggagcttataaggggaggtgaactccctatcccagatggggccaatatggatgaactattacaaggcgtactgggattggaaggtatcgtgaggcgtagggatatgtccatcagaagcgccaagtccatccaagatccatttcttcaattcgaagtgaaaatgagcaaaaacttgcccagaggaagagctctcatcctgaacactacagaatcgatagactctctttctttgcgacacattcggtcgatctgtcccactacctacgcactcgggcccttccacgtccttctcaggaacataaaagacgagtcccactccgcaagcctttccgaagaggacaggtcctgcatcgcctggctggactcgaaaccgaacaagtccgcggtctacgtgagtttcggtagcctcgccgccatggcgagagaagcatttcttgagtttcagcagggattgctcgacagcgggtattacttcttgtgggtgatccggcccgatatggtggaaggggggctggaagagagcgagctgaccgcgagcgaacaacgctactttgtgaagtgggccccacaggaggaggttcttgcgcacccggcggtagggtgtttcttgacgcacagcggttggaactctacgttggagagtatctttgcgggagtgccgatgatatgttggcctttctttgcggaccagctgattaacagtaggtttgcgagcgaggtgtggaaaattgccttggatatgaaggatttgtgcggaaggagccacgtggagaggatggtgaaggaagttatgagtggagagaaaggcgaagagctaaggaattctagctgcgagatggcagatagggtgaagaagagtgcagaggaaggtggctcttcctacgccaacttcaaagagttggttggacatatcaaatctttgagcttaccagcagaaagaggagaaaatggtggtgaaggaatgagtgtacaagcgccgagtaaacttttcctcctcaacgctgaggacggaaaacatgtccttaaaagtgacgaaccgtcggaacaaaggggtccacaatttaatccaaattttcttcggacctgagcttcggccatgctagagtccgcaaaaatcaccagtctctctctacaaatctatctctctctatttttctccagaataatgtgtgagtagttcccagataagggaattagggttcttatagggtttcgctcatgtgttgagcatataagaaacccttagtatgtatttgtatttgtaaaatacttctatcaataaaatttctaattcctaaaaccaaaatccagtgacctcgctgtcaggagagcgcgagtcggtcccattattgaagcatttatcagggttattgtctcatgagcggatacatatttgaatgtatttagaaaaataaacaaataggggttccgcgcacatttccccgaaaagtgccacctgacgtctaagaaaccattattatcatgacattaacctataaaaataggcgtatcacgaggccctttcgtcttcaagaattagcttggcaattcccgatctagtaacatagatgacaccghgcgcgataatttatcctagtttgcgcgctatattttgttttctatcgcgtattaaatgtataattgcgggactctaatcataaaaacccatctcataaataacgtcatgcattacatgttaattattacatgcttaacgtaattcaacagaaattatatgataatcgtcgcaagaccggcaacaggattcaatcttaagaaactttattgccaaatgtttgaacgatcgggatcgaagatccattccaagctcattcctttgccctcggacgagtgctggggcgtcggtttccactatcggcgagtacttctacacagccatcggtccagacggccgcgcttctgcgggcgatttgtgtacgcccgacagtcccggctccggatcggacgattgcgtcgcatcgaccctgcgcccaagctgcatcatcgaaattgccgtcaaccaagctctgatagagttggtcaagaccaatgcggagcatatacgcccggagtcgtggcgatcctgcaagctccggatgcctccgctcgaagtagcgcgtctgctgctccatacaagccaaccacggcctccagaagaagatgttggcgacctcgtattgggaatccccgaacattgcctcgctccagtcaatgaccgctgttatgcggccattgtccgtcaggacattgttggagccgaaatccgcgtgcacgaggtgccggacttcggggcagtcctcggcccaaagcatcagctcatcgagagcctgcgcgacggacgcactgacggtgtcgtccatcacagtttgccagtgatacacatggggatcagcaatcgcgcatatgaaatcacgccatgtagtgtattgaccgattccttgcggtccgaatgggccgaacccgctcgtctggctaagatcggccgcagcgatcgcatccatggcctccgcgaccggctgcagaacagcgggcagttcggtttcaggcaggtcttgcaacgtgacaccctgtgcacggcgggagatgcaataggtcaggctctcgctgaattccccaatgtcaagcacttccggaatcgggagcgcggccgatgcaaagtgccgataaacataacgatctttgtagaaaccatcggcgcagctatttacccgcaggacatatccacgccctcctacatcgaagctgaaagcacgagattcttcgccctccgagagctgcatcaggtcggacacgctgtcgaacttttcgatcagaaacttctcgacagacgtcgcggtgagttcaggctttttcattgcctcgatcgagttgagagtgaatatgagactctaattggataccgaggggaatttatggaacgtcagtggagcatttttgacaagaaatatttgctagctgatagtgaccttaggcgacttttgaacgcgcaataatggtttctgacgtatgtgcttagctcattaaactccagaaacccgcggctcagtggctccttcaacgttgcggttctgtcagttccaaacgtaaaacggcttgtcccgcgtcatcggcgggggtcataccgtgactcccttaattctcatgtatctccgtcaggagtccctaatgatattgttcacgtaattaagttttgtggaagtgagagagtccaattttgataagaaaagagtcagaaaacgtaatattttaaaagtctaaatctttctacaaataagagcaaatttatttattttttaatccaataaatattaatggaggacaaattcaattcacttggttgtaaaataaacttaaaccaataaccaaagaactaataaatcctgaagtggaattattaaggataaatgtacatagacaatgaagaaataataggttcgatgaattaataataattaaggatgttacaatcatcatgtgccaagtatatacacaatattctatgggatttataatttcgttacttcacttaacttttgcgtaaataaaacgaattatctgatattttataataaaacagttataagaaccatcatttttaacaacatagatatattatttctaatagtttaatgatacttttaaatcttttaaattttatgtttcttttagaaaataaaaattcaaaaaattaaatatatttacaaaaactacaatcaaacacaacttcatatattaaaagcaaaatatattttgaaaatttcaagtgtcctaacaaataagacaagaggaaaatgtacgatgagagacataaagagaactaataattgaggagtcctataatatataataaagtttattagtaaacttaattattaaggactcctaaaatatatgataggagaaaatgaatggtgagagatattggaaaacttaataattaaggattttaaaatatatggtaaaagataggcaaagtatccattatccccttttaacttgaagtctactaggcgcatgtgaaagttgattttttgtcacgtcatatagctataacgtaaaaaaagaaagtaaaatttttaattttttttaatatatgacatattttaaacgaaatataggacaaaatgtaaatgaatagtaaaggaaacaaagattaatacttactttgtaagaatttaagataaatttaaaatttaatagatcaactttacgtctagaaagacccatatctagaaggaatttcacgaaatcggcccttattcgaaaataacttttaaataatgaattttaaattttaagaaataatatccaatgaataaatgacatgtagcattttacctaaatatttcaactattttaatccaatattaatttgttttattcccaacaatagaaagtcttgtgcagacatttaatctgacttttccagtactaaatattaattttctgaagattttcgggtttagtccacaagttttagtgagaagttttgctcaaattttaggtgagaaggtttgatatttatcttttgttaaattaatttatctaggtgactattatttatttaagtagaaattcatatcattacttttgccaacttgtagtcataataggagtaggtgtatatgatgaaggaataaacaagttcagtgaagtgattaaaataaaatataatttaggtgtacatcaaataaaaaccttaaagtttagaaaggcaccgaataattttgcatagaagatattagtaaatttataaaaataaaagaaatgtagttgtcaagttgtcttcttttttttggataaaaatagcagttggcttatgtcattcttttacaacctccatgccacttgtccaattgttgacacttaactaattagtttgattcatgtatgaatactaaataattttttaggactgactcaaatatttttatattatcatagtaatatttatctaatttttaggaccacttattactaaataataaattaactacaactatattattgttgtgaaacaacaacgttttggttgttatgatgaaacgtacactatatcagtatgaaaaattcaaaacgattagtataaattatattgaaaatttgatatttttctattcttaatcagacgtattgggtttcatattttaaaaagggactaaacttagaagagaagtttgtttgaaactacttttgtctctttcttgttcccatttctctcttagatttcaaaaagtgaactactttatctccttctttgttcacattttattttattctattataaatatggcatcctcatattgagatttttagaaattattctaatcattcacagtgcaaaagaagaatggaatctcctgctactaaattacctgcacctctgctgatgttatcttcttctccattccttctcccttctcctaataagagctcctccatcttccttccacgtaaattagggccgctacctccaaaatattattattacaattgctgccatcctaagagtagatcaatctcagtagtatcaatggcaaataaggaggaggcagagacaagtaagaagaagcccaaaccattaaaagtactaattaccaaagtggatccgaagccgaggaagggcatggcatccgtcgcagtggacttactcgagaaggcctttgtatacctattgtccggaaattctgcagctgatcgtagtagtagtagtggtcgtcgtcgtcgtaaagagcattactacctctccggcaattatgcgcccgtcggacacgaaaccccgccctccgaccacctccccattcatggatcccttcctgaatgcttgaatggagtgtttctgagagttggtcctaaccccaagtttgctcccgtagccggatacaattgggtcgatggagatggaatgattcatggattgcgtattaaagatggaaaagcaacttatctatctcgatatattaaaacgtcacggtttaaacaagaagaatattttggaagagcaaaatttatgaagattggagatctaaggggattgcttgggttctttacgatcttaatactagtacttcgaacaacattgaaagtaatagacatttcatatggaagagggacgggtaatacagctcttgtgtatcataatggcttactattggctctatcagaagaagataaaccttatgttgttaaagttttagaagatggagacttgcaaactcttgggatattggattatgacaagaaattgtcacatccattcaccgctcatccaaagatcgatccgttaactgatgagatgtttacctttggatattccatctcgcctccgtatcttacttatcgagtcatttccaaggatggagtgatgcaagatccagtgcaaatctcaattacatcccctaccataatgcatgattttgctattactgaaaattatgccatcttcatggacctgcccttgtatttccaaccagaggaaatggtaaaggggaaatttgtctcttcatttcaccctacaaaaagagctcgtatcggtgtgcttccacgatatgcaaaagacgagcatccaattcgatggttcgatcttccaagttgcttcatgactcataatgcaaatgcttgggaagagaatgatgaagttgtgctattcacatgtcgccttgagagtcctgatcttgacatgcttagtggacctgcggaagaagagattgggaattcaaaaagtgagctttacgaaatgaggttcaatttgaaaactggaattacttcacaaaagcaactatctgtacctagtgttgattttcctcggatcaaccaaagttatactggcaggaaacagcaatatgtttattgtactcttggcaacaccaagattaagggcattgtgaagtttgatctgcaaattgaaccagaagccggaaagacaatgcttgaagttggaggaaatgtacaaggcatctttgagttgggacctagaagatatggttcagaggcaatatttgtgccatgccaacctggcatcaaatctgatgaggatgacggttacttgatattctttgtacacgacgaaaacaatgggaaatctgaggtcaatgtcatcgatgcaaagacaatgtctgcagaacctgtggctgttgtggaacttccaagcagggttccatatggattccatgccttgtttctgaatgaggaagaacttcagaagcaccaagcagagacatgagcttcggccatgctagagtccgcaaaaatcaccagtctctctctacaaatctatctctctctatttttctccagaataatgtgtgagtagttcccagataagggaattagggttcttatagggtttcgctcatgtgttgagcatataagaaacccttagtatgtatttgtatttgtaaaatacttctatcaataaaatttctaattcctaaaaccaaaatccagtgacctcgctgtcatgagacgaattctgacaggatatattggcgggtaaacctaagagaaaagagcgtttattagaataatcggatatttaaaagggcgtgaaaaggtttatccgttcgtccatttgtatgtgcatgccaaccacagggttcccctcgggatcaaagtactttgatccaacccctccgctgctatagtgcagtcggcttctgacgttcagtgcagccgtcatctgaaaacgacatgtcgcacaagtcctaagttacgcgacaggctgccgccctgcccttttcctggcgttttcttgtcgcgtgttttagtcgcataaagtagaatacttgcgactagaaccggagacattacgccatgaacaagagcgccgccgctggcctgctgggctatgcccgcgtcagcaccgacgaccaggacttgaccaaccaacgggccgaactgcacgcggccggctgcaccaagctgttttccgagaagatcaccggcaccaggcgcgaccgcccggagctggccaggatgcttgaccacctacgccctggcgacgttgtgacagtgaccaggctagaccgcctggcccgcagcacccgcgacctactggacattgccgagcgcatccaggaggccggcgcgggcctgcgtagcctggcagagccgtgggccgacaccaccacgccggccggccgcatggtgttgaccgtgttcgccggcattgccgagttcgagcgttccctaatcatcgaccgcacccggagcgggcgcgaggccgccaaggcccgaggcgtgaagtttggcccccgccctaccctcaccccggcacagatcgcgcacgcccgcgagctgatcgaccaggaaggccgcaccgtgaaagaggcggctgcactgcttggcgtgcatcgctcgaccctgtaccgcgcacttgagcgcagcgaggaagtgacgcccaccgaggccaggcggcgcggtgccttccgtgaggacgcattgaccgaggccgacgccctggcggccgccgagaatgaacgccaagaggaacaagcatgaaaccgcaccaggacggccaggacgaaccgtttttcattaccgaagagatcgaggcggagatgatcgcggccgggtacgtgttcgagccgcccgcgcacctctcaaccgtgcggctgcatgaaatcctggccggtttgtctgatgccaagctggcggcctggccggccagcttggccgctgaagaaaccgagcgccgccgtctaaaaaggtgatgtgtatttgagtaaaacagcttgcgtcatgcggtcgctgcgtatatgatccgatgagtaaataaacaaatacgcaaggggaacgcatgaaggttatcgctgtacttaaccagaaaggcgggtcaggcaagacgaccatcggaacccatctagcccgcgccctgcaactcgccggggccgatgttctgttagtcgattccgatccccagggcagtgcccgcgattgggcggccgtgcgggaagatcaaccgctaaccgttgtcggcatcgaccgcccgacgattgaccgcgacgtgaaggccatcggccggcgcgacttcgtagtgatcgacggagcgccccaggcggcggacttggctgtgtccgcgatcaaggcagccgacttcgtgctgattccggtgcagccaagcccttacgacatatgggccaccgccgacctggtggagctggttaagcagcgcattgaggtcacggatggaaggctacaagcggcctttgtcgtgtcgcgggcgatcaaaggcacgcgcatcggcggtgaggttgccgaggcgctggccgggtacgagctgcccattcttgagtcccgtatcacgcagcgcgtgagctacccaggcactgccgccgccggcacaaccgttcttgaatcagaacccgagggcgacgctgcccgcgaggtccaggcgctggccgctgaaattaaatcaaaactcatttgagttaatgaggtaaagagaaaatgagcaaaagcacaaacacgctaagtgccggccgtccgagcgcacgcagcagcaaggctgcaacgttggccagcctggcagacacgccagccatgaagcgggtcaactttcagttgccggcggaggatcacaccaagctgaagatgtacgcggtacgccaaggcaagaccattaccgagctgctatctgaatagatcgcgcagctaccagagtaaatgagcaaatgaataaatgagtagatgaattttagcggctaaaggaggcggcatggaaaatcaagaacaaccaggcaccgacgccgtggaatgccccatgtgtggaggaacgggcggttggccaggcgtaagcggctgggttgtctgccggccctgcaatggcactggaacccccaagcccgaggaatcggcgtgacggtcgcaaaccatccggcccggtacaaatcggcgcggcgctgggtgatgacctggtggagaagttgaaggccgcgcaggccgcccagcggcaacgcatcgaggcagaagcacgccccggtgaatcgtggcaagcggccgctgatcgaatccgcaaagaatcccggcaaccgccggcagccggtgcgccgtcgattaggaagccgcccaagggcgacgagcaaccagattttttcgttccgatgctctatgacgtgggcacccgcgatagtcgcagcatcatggacgtggccgttttccgtctgtcgaagcgtgaccgacgagctggcgaggtgatccgctacgagcttccagacgggcacgtagaggtttccgcagggccggccggcatggccagtgtgtgggattacgacctggtactgatggcggtttcccatctaaccgaatccatgaaccgataccgggaagggaagggagacaagcccggccgcgtgttccgtccacacgttgcggacgtactcaagttctgccggcgagccgatggcggaaagcagaaagacgacctggtagaaacctgcattcggttaaacaccacgcacgttgccatgcagcgtacgaagaaggccaagaacggccgcctggtgacggtatccgagggtgaagccttgattagccgctacaagatcgtaaagagcgaaaccgggcggccggagtacatcgagatcgagctagctgattggatgtaccgcgagatcacagaaggcaagaacccggacgtgctgacggttcaccccgattactttttgatcgatcccggcatcggccgttttctctaccgcctggcacgccgcgccgcaggcaaggcagaagccagatggttgttcaagacgatctacgaacgcagtggcagcgccggagagttcaagaagttctgtttcaccgtgcgcaagctgatcgggtcaaatgacctgccggagtacgatttgaaggaggaggcggggcaggctggcccgatcctagtcatgcgctaccgcaacctgatcgagggcgaagcatccgccggttcctaatgtacggagcagatgctagggcaaattgccctagcaggggaaaaaggtcgaaaaggactctttcctgtggatagcacgtacattgggaacccaaagccgtacattgggaaccggaacccgtacattgggaacccaaagccgtacattgggaaccggtcacacatgtaagtgactgatataaaagagaaaaaaggcgatttttccgcctaaaactctttaaaacttattaaaactcttaaaacccgcctggcctgtgcataactgtctggccagcgcacagccgaagagctgcaaaaagcgcctacccttcggtcgctgcgctccctacgccccgccgcttcgcgtcggcctatcgcggccgctggccgctcaaaaatggctggcctacggccaggcaatctaccagggcgcggacaagccgcgccgtcgccactcgaccgccggcgcccacatcaaggcaccctgcctcgcgcgtttcggtgatgacggtgaaaacctctgacacatgcagctcccggtgacggtcacagcttgtctgtaagcggatgccgggagcagacaagcccgtcagggcgcgtcagcgggtgttggcgggtgtcggggcgcagccatgacccagtcacgtagcgatagcggagtgtatactggcttaactatgcggcatcagagcagattgtactgagagtgcaccatatgcggtgtgaaataccgcacagatgcgtaaggagaaaataccgcatcaggcgctcttccgcttcctcgctcactgactcgctgcgctcggtcgttcggctgcggcgagcggtatcagctcactcaaaggcggtaatacggttatccacagaatcaggggataacgcaggaaagaacatgtgagcaaaaggccagcaaaaggccaggaaccgtaaaaaggccgcgttgctggcgtttttccataggctccgcccccctgacgagcatcacaaaaatcgacgctcaagtcagaggtggcgaaacccgacaggactataaagataccaggcgtttccccctggaagctccctcgtgcgctctcctgttccgaccctgccgcttaccggatacctgtccgcctttctcccttcgggaagcgtggcgctttctcatagctcacgctgtaggtatctcagttcggtgtaggtcgttcgctccaagctgggctgtgtgcacgaaccccccgttcagcccgaccgctgcgccttatccggtaactatcgtcttgagtccaacccggtaagacacgacttatcgccactggcagcagccactggtaacaggattagcagagcgaggtatgtaggcggtgctacagagttcttgaagtggtggcctaactacggctacactagaaggacagtatttggtatctgcgctctgctgaagccagttaccttcggaaaaagagttggtagctcttgatccggcaaacaaaccaccgctggtagcggtggtttttttgtttgcaagcagcagattacgcgcagaaaaaaaggatctcaagaagatcctttgatcttttctacggggtctgacgctcagtggaacgaaaactcacgttaagggattttggtcatgcattctaggtgattagaaaaactcatcgagcatcaaatgaaactgcaatttattcatatcaggattatcaataccatatttttgaaaaagccgtttctgtaatgaaggagaaaactcaccgaggcagttccataggatggcaagatcctggtatcggtctgcgattccgactcgtccaacatcaatacaacctattaatttcccctcgtcaaaaataaggttatcaagtgagaaatcaccatgagtgacgactgaatccggtgagaatggcaaaagtttatgcatttctttccagacttgttcaacaggccagccattacgctcgtcatcaaaatcactcgcatcaaccaaaccgttattcattcgtgattgcgcctgagcgagtcgaaatacgcgatcgctgttaaaaggacaattacaaacaggaatcgaatgcaaccggcgcaggaacactgccagcgcatcaacaatattttcacctgaatcaggatattcttctaatacctggaatgctgttttccctgggatcgcagtggtgagtaaccatgcatcatcaggagtacggataaaatgcttgatggtcggaagaggcataaattccgtcagccagtttagtctgaccatctcatctgtaacatcattggcaacgctacctttgccatgtttcagaaacaactctggcgcatcgggcttcccatacaatcggtagattgtcgcacctgattgcccgacattatcgcgagcccatttatacccatataaatcagcatccatgttggaatttaatcgcggccttgagcaagacgtttcccgttgaatatggctcataacagaacttattatttccttcctcttttctacagtatttaaagataccccaagaagctaattataacaagacgaactccaattcactgttccttgcattctaaaaccttaaataccagaaaacagctttttcaaagttgttttcaaagttggcgtataacatagtatcgacggagccgattttgaaaccgcggtgatcacaggcagcaacgctctgtcatcgttacaatcaacatgctaccctccgcgagatcatccgtgtttcaaacccggcagcttagttgccgttcttccgaatagcatcggtaacatgagcaaagtctgccgccttacaacggctctcccgctgacgccgtcccggactgatgggctgcctgtatcgagtggtgattttgtgccgagctgccggtcggggagctgttggctggctggtggcaggatatattgtggtgtaaacataacgaattcgtctca

SEQ ID NO: 22 - DNA, 20976 bp, synthetic construct
  source 1..20976: mol_type = other DNA; plasmid = DNA construct O2 = pDGB3alpha1[p2A11:UGT2:T35S-p35S:UGT709G1:T35S-pE8:CCD2L:T35S-pNos:Hyg:T35S]
ggaggtcaaacaattttgaggaattcaatttcatctttaactggtacaataatcattttatcatgaaaataagcagctcaagagaatttttgaagaatcttttatttctttaacatttaaccacatgaatttttaatttttttttgcaatacatttaaaccgaaatggtcaaacgatcaaccaactgatctttattctaataaacttctagtttacatttgcatgtgagtgcatcatcattatcatatttgtacacaacaaacaagaaaaaaatataaacaatattttatttaaatatttatattccactttgactgtagatattaaatcttgtcatcatttatagtctcaatattataatttttttattttttcaaaattcaaaagtttacaattatttttttgaactataatattatccaagatgaacatctcaagaagaaaattattaatattgttatggttaaaattttacatacaatacttgttttttgctttacttttatcttaccgtagatacacaatcgacgataacttagtgatcacacaataataattattttgttcatgacacaatatttataagaaatacttatttctttcttttatccttcagtagttcataataaaaacataccataatatttgtgatgcattcatagtacgtaatgaaatgacaatttatgtcaaattattttcttttatactctcaaacctcccgtaaaggtgagatgagtcatttatccaattatacataaatatgtctttattcatgctctttatcacattctgacacattcacttaatttcaagagtaagcaagcatgataactgaaactatttatgcgtatcttaccttgatatttgacacattacatgacacacctcaacatcactttcaaagattaagcgcaccaccatattatctttctttttttttttatgaaggttttataaaattattaaattaggtccaaaaaattgtttgtcaaataaccttttatactagattgatgacaaaaattacctttacgttttgaaagaccattttaagacctaatctatcagtgactccttaaagttggcacaatatttcacttagacaccctaattgaatgatgttcattttaaacacccaatgtagggttccgctatatcattttgacacatttcttaacatcaacaaaaatatataatgagtatgtgatatactcgcgaatgacgtgaaaaatgaagacatttgttatttgtatcaaagtagttactaaataattaattttgaataaaaataaaagctgaccagtaaatcaataacacataatattttccacctaataattaaaatataaaataaaaaagagccatctcagggtcatctgcccaccattgctatttcaaagaaatttgtacgttagtttatagaaattgatgttaaaattctttcaagaaaaatttatgaatgaatttattctctaatttaaaaatattttctgttatttttgttgaaagaaatttaacttggataaaatggtggttaaaactggaaagaagaaaagagaaaaaataattaaaaatcatttcacgctctaatcaatgagcgtatcacattcattatgttatataagcaaaagtgacaaaacgaaaataatatattacatgaaatgtctaaaataaatatcgtctaattaaaatatctaagtaacatattgtgcctaactttagagggatcatcaataagttaaaccccattttaataactcataattgtcctttttatttaatattgtcacaaatcacaatgataattaacattaatttgtcctttgtgacgtccatattcatgcatttaaccaatcatcttcatttggacttattatcacaattatcccactttcctcacaaaatggagcattcaagtggaatagactacacgatttttaatttcatcaaaaacatctttttgctttattcattattatattgtcgctattgttgaattttatttgccctaaatttcttaccataaatagatttttcttttagaaaaaggagattgactaattcttttcttgtaggaaaaggtttaggactctataaatagagacatattccttctaacttaatcaacatttacaatgtagtcttaaagactttgaaagtttttggttagggggagaaattgtgggtcacaagcttgatacgttatcaattgtgtaaacctcccatgtattctgagtgaatttggttgaggttgtttccctctgtattttgtactctcatatttatagtggattgttcatctctttcgtggacgtaggtcgattgaccgtcgattgaccgaaccacgttaaatctttgtattttttgatatatttctcattatcttcttactcgtgatctttcaaggtttgcattgctatcttccgcgttacaccaacttatttacgatcctaacagctatggtgtggaaacataaatcaaacattttactgatataaacacatctttgattataacatgatagaaatttgagcccaactttttatcatcattatatacaaaaagttctaaattttttttttgatgtagtaaaacttaaatccatagtcttgcccctaaaccaatgacataatatataacccaaaatatactagttttcgccctcgagccctttaaaaagtatagtcaatatttacggtgaccgtgaatttcttaattatgatatataatttaaaagaaatcatgatcacattctactgatgagaacatgtgctaatcaagggaaaacatggatgtgaaaaatactttttgttaaaagtaaaaaaaaatgtgaaattttgttagttatttactacctatacattatttgagcatgtgcaaactttacaaatacctaatagaagattttcacctgcctgtatatatgtaaattaattataatgaacactctcacataaaataattatcagtatatacattaatacttgccctccacaatgaattaaataaaatgtagaacatgatctacacttcaataaaactaagaccataaagaataatttcaaaatatacacatgtcaacaataaattatttgcatattatattaacttactaaacaatctttacttttgaaatataaaaataatcaagttataagtctgctcaaagtaaagcacttgttagactcatctgattttgagaaggtaagcaaattgatggtgcataatagtcacaagtaaaatataaaatagatttcattagtaaaattgttttttactttctttatatataattatcaatatccttcaatggtaggttaattatattgttaacttcttgttgaattaaagcaataagacaagaatattaaagataaaagaacaataaaaatagaaagactaagagataagagttttcttattcttctttcaataagtatcatcaagtgtatacaatataaatttttgtatttttgatctatctatttataatgttatatataagcatacaaaagatcagtcataaatatgactttaatcatgaaaataatgaaagagattatgaaggcgtaaggttactagaataatagtcattaaaaaaaggggttatctttataattgaataattgatgaagtaatggagataattagtgagcataaatttttttaaaaaaatggacatttacactataatattttataacactttcccttaaacatctaggtataaataatgagtcttgtcaaaatcttagtaggaaaaattctgtgaaatttttttagtgaaaacaaatgatataaatatcttgaatactcattatttgttgtctcattaaaaatcttatctgacctataaaataaattatttgctcaactcaaaatagtttttcattctaaaattagtataattattagtgaatatttaattaacataattgtatactaaggggcctataaattggattcttctcaaagaaaaataaaatcaccacacaactttcttcttctgctcatcaattagcaattaatccaaaaccaaatgttgaacggcaacaaatgccacatcctcctcctcccctgtccagcacaaggccatatcaaccccattctccaattcggcaagcgactggcctctcacaacctcctcaccacactcgtcaacacccggttcctctccaactcgaccaaatccgaacccggtccggtcaacatccagtgcatatccgacggattcgatcccggtgggatgaatgcagcacctagtcgtcgggcctatttcgaccgacctcagagtcggtcgggtcagaaacatgttggcctcatcgagtcactccggtccagaggccgacccggcgcatgttttggtctacgacccgttcccctctgggcaatgaacgtagccgagcggtccgggctgcggtcggtcgcattctttactcagccgtgtgcagtggacacaatctaccgccacgtgtgggagggacgaattaaggttccggttgccgagccggtccggttgcctggattgcccccactcgagcctagtgatctgccgtgcgttcgtaacggattcggacgagtcgttaacccggatctcttgccacttcgagtgaatcagcacaaaaatttggacaaagctgacatgatggggaggaactccatatacgagctagaggcggatttgttggatgggtcccgattaccattaccggtgaagtcgattgggccgaccgtgccgtctacttatctcgacaaccgaatcccgtcggattcacactatggattcaatctatacacccctgacactactccctacttggactggctcgactccaaggccccgaactctgtcatctatgtctcatttggtagtttgtccagtctgagccctgatcaaaccaatgagattgcgtcgggtctgatcgccaccaacaaaagctttatttgggtggtacgcacttcggagttagccaaactccctgccaacttcacccaagagaatgcgagccgtgggctggttgtgacctggtgcgaccaactcgatctcctcgcacacgttgcgaccggttgcttcgtgactcactgcggatggaactcgactatggaaggtgtcgcacttggtgtgccgatggtgggagtgccgcagtggtcggaccagcctatgaatgccaagtatgtagaggatgtgtggaaggtcggcgtgagggcgaagacttatgggaaggattttgtgagaggggaggagttcaaaagatgtgtggaggaggtgatggatggagagaggagtggaaagattagagagaatgccgcaaggtggtgtaagttggccaaggactctgttagtgagggtgggagttctgacaagtgtatcaaggagttcatacatcagtgttgcaatgactccaaaatttccttagtttaagcttcggccatgctagagtccgcaaaaatcaccagtctctctctacaaatctatctctctctatttttctccagaataatgtgtgagtagttcccagataagggaattagggttcttatagggtttcgctcatgtgttgagcatataagaaacccttagtatgtatttgtatttgtaaaatacttctatcaataaaatttctaattcctaaaaccaaaatccagtgacctcgctgtcaggagactagagccaagctgatctcctttgccccggagatcaccatggacgactttctctatctctacgatctaggaagaaagttcgacggagaaggtgacgataccatgttcaccaccgataatgagaagattagcctcttcaatttcagaaagaatgctgacccacagatggttagagaggcctacgcggcaggtctgatcaagacgatctacccgagtaataatctccaggagatcaaataccttcccaagaaggttaaagatgcagtcaaaagattcaggactaactgcatcaagaacacagagaaagatatatttctcaagatcagaagtactattccagtatggacgattcaaggcttgcttcataaaccaaggcaagtaatagagattggagtctctaagaaagtagttcctactgaatcaaaggccatggagtcaaaaattcagatcgaggatctaacagaactcgccgtgaagactggcgaacagttcatacagagtcttttacgactcaatgacaagaagaaaatcttcgtcaacatggtggagcacgacactctcgtctactccaagaatatcaaagatacagtctcagaagaccaaagggctattgagacttttcaacaaagggtaatatcgggaaacctcctcggattccattgcccagctatctgtcacttcatcaaaaggacagtagaaaaggaaggtggcacctacaaatgccatcattgcgataaaggaaaggctatcgttcaagatgcctctgccgacagtggtcccaaagatggacccccacccacgaggagcatcgtggaaaaagaagacgttccaaccacgtcttcaaagcaagtggattgatgtgatatctccactgacgtaagggatgacgcacaatcccactatccttcgcaagacccttcctctatataaggaagttcatttcatttggagaggactccggtatttttacaacaataccacaacaaaacaaacaacaaacaacattacaatttactattctagtcgaaatggctgagaaagaagcaaatacccatgtcgtcctcttccccttgccaggccaagggcacatcggctcaatgttgaaactggcacagcttctttccaccgccggattctacgtcactttcgtccacaccgaacgcaactaccgtcgctacctcctcacctccacgtccttccacgtccccaagttccggttccgcaccatccccgacggttttcccgacgacgattcccgctcgcccctcccttttctcgagctccaagagtcgctggacacgaaatgtcgggggcattatcgggaattgttggtcgctgtcgacgaccaagaagagtggcccccagtcacttgtgtcgtggctgatcaagctcttccactctcactcgaagttcccgacgagttggggattcctgtaatgatactcgcaccacacagtgcgtgcagtatattgacgagttattcgattccggagcttataaggggaggtgaactccctatcccagatggggccaatatggatgaactattacaaggcgtactgggattggaaggtatcgtgaggcgtagggatatgtccatcagaagcgccaagtccatccaagatccatttcttcaattcgaagtgaaaatgagcaaaaacttgcccagaggaagagctctcatcctgaacactacagaatcgatagactctctttctttgcgacacattcggtcgatctgtcccactacctacgcactcgggcccttccacgtccttctcaggaacataaaagacgagtcccactccgcaagcctttccgaagaggacaggtcctgcatcgcctggctggactcgaaaccgaacaagtccgcggtctacgtgagtttcggtagcctcgccgccatggcgagagaagcatttcttgagtttcagcagggattgctcgacagcgggtattacttcttgtgggtgatccggcccgatatggtggaaggggggctggaagagagcgagctgaccgcgagcgaacaacgctactttgtgaagtgggccccacaggaggaggttcttgcgcacccggcggtagggtgtttcttgacgcacagcggttggaactctacgttggagagtatctttgcgggagtgccgatgatatgttggcctttctttgcggaccagctgattaacagtaggtttgcgagcgaggtgtggaaaattgccttggatatgaaggatttgtgcggaaggagccacgtggagaggatggtgaaggaagttatgagtggagagaaaggcgaagagctaaggaattctagctgcgagatggcagatagggtgaagaagagtgcagaggaaggtggctcttcctacgccaacttcaaagagttggttggacatatcaaatctttgagcttaccagcagaaagaggagaaaatggtggtgaaggaatgagtgtacaagcgccgagtaaacttttcctcctcaacgctgaggacggaaaacatgtccttaaaagtgacgaaccgtcggaacaaaggggtccacaatttaatccaaattttcttcggacctgagcttcggccatgctagagtccgcaaaaatcaccagtctctctctacaaatctatctctctctatttttctccagaataatgtgtgagtagttcccagataagggaattagggttcttatagggtttcgctcatgtgttgagcatataagaaacccttagtatgtatttgtatttgtaaaatacttctatcaataaaatttctaattcctaaaaccaaaatccagtgacctcgctgtcaggagagcgcgagtcggtcccattattgaagcatttatcagggttattgtctcatgagcggatacatatttgaatgtatttagaaaaataaacaaataggggttccgcgcacatttccccgaaaagtgccacctgacgtctaagaaaccattattatcatgacattaacctataaaaataggcgtatcacgaggccctttcgtcttcaagaattagcttggcaattcccgatctagtaacatagatgacaccghgcgcgataatttatcctagtttgcgcgctatattttgttttctatcgcgtattaaatgtataattgcgggactctaatcataaaaacccatctcataaataacgtcatgcattacatgttaattattacatgcttaacgtaattcaacagaaattatatgataatcgtcgcaagaccggcaacaggattcaatcttaagaaactttattgccaaatgtttgaacgatcgggatcgaagatccattccaagctcattcctttgccctcggacgagtgctggggcgtcggtttccactatcggcgagtacttctacacagccatcggtccagacggccgcgcttctgcgggcgatttgtgtacgcccgacagtcccggctccggatcggacgattgcgtcgcatcgaccctgcgcccaagctgcatcatcgaaattgccgtcaaccaagctctgatagagttggtcaagaccaatgcggagcatatacgcccggagtcgtggcgatcctgcaagctccggatgcctccgctcgaagtagcgcgtctgctgctccatacaagccaaccacggcctccagaagaagatgttggcgacctcgtattgggaatccccgaacattgcctcgctccagtcaatgaccgctgttatgcggccattgtccgtcaggacattgttggagccgaaatccgcgtgcacgaggtgccggacttcggggcagtcctcggcccaaagcatcagctcatcgagagcctgcgcgacggacgcactgacggtgtcgtccatcacagtttgccagtgatacacatggggatcagcaatcgcgcatatgaaatcacgccatgtagtgtattgaccgattccttgcggtccgaatgggccgaacccgctcgtctggctaagatcggccgcagcgatcgcatccatggcctccgcgaccggctgcagaacagcgggcagttcggtttcaggcaggtcttgcaacgtgacaccctgtgcacggcgggagatgcaataggtcaggctctcgctgaattccccaatgtcaagcacttccggaatcgggagcgcggccgatgcaaagtgccgataaacataacgatctttgtagaaaccatcggcgcagctatttacccgcaggacatatccacgccctcctacatcgaagctgaaagcacgagattcttcgccctccgagagctgcatcaggtcggacacgctgtcgaacttttcgatcagaaacttctcgacagacgtcgcggtgagttcaggctttttcattgcctcgatcgagttgagagtgaatatgagactctaattggataccgaggggaatttatggaacgtcagtggagcatttttgacaagaaatatttgctagctgatagtgaccttaggcgacttttgaacgcgcaataatggtttctgacgtatgtgcttagctcattaaactccagaaacccgcggctcagtggctccttcaacgttgcggttctgtcagttccaaacgtaaaacggcttgtcccgcgtcatcggcgggggtcataccgtgactcccttaattctcatgtatctccgtcaggagtccctaatgatattgttcacgtaattaagttttgtggaagtgagagagtccaattttgataagaaaagagtcagaaaacgtaatattttaaaagtctaaatctttctacaaataagagcaaatttatttattttttaatccaataaatattaatggaggacaaattcaattcacttggttgtaaaataaacttaaaccaataaccaaagaactaataaatcctgaagtggaattattaaggataaatgtacatagacaatgaagaaataataggttcgatgaattaataataattaaggatgttacaatcatcatgtgccaagtatatacacaatattctatgggatttataatttcgttacttcacttaacttttgcgtaaataaaacgaattatctgatattttataataaaacagttataagaaccatcatttttaacaacatagatatattatttctaatagtttaatgatacttttaaatcttttaaattttatgtttcttttagaaaataaaaattcaaaaaattaaatatatttacaaaaactacaatcaaacacaacttcatatattaaaagcaaaatatattttgaaaatttcaagtgtcctaacaaataagacaagaggaaaatgtacgatgagagacataaagagaactaataattgaggagtcctataatatataataaagtttattagtaaacttaattattaaggactcctaaaatatatgataggagaaaatgaatggtgagagatattggaaaacttaataattaaggattttaaaatatatggtaaaagataggcaaagtatccattatccccttttaacttgaagtctactaggcgcatgtgaaagttgattttttgtcacgtcatatagctataacgtaaaaaaagaaagtaaaatttttaattttttttaatatatgacatattttaaacgaaatataggacaaaatgtaaatgaatagtaaaggaaacaaagattaatacttactttgtaagaatttaagataaatttaaaatttaatagatcaactttacgtctagaaagacccatatctagaaggaatttcacgaaatcggcccttattcgaaaataacttttaaataatgaattttaaattttaagaaataatatccaatgaataaatgacatgtagcattttacctaaatatttcaactattttaatccaatattaatttgttttattcccaacaatagaaagtcttgtgcagacatttaatctgacttttccagtactaaatattaattttctgaagattttcgggtttagtccacaagttttagtgagaagttttgctcaaattttaggtgagaaggtttgatatttatcttttgttaaattaatttatctaggtgactattatttatttaagtagaaattcatatcattacttttgccaacttgtagtcataataggagtaggtgtatatgatgaaggaataaacaagttcagtgaagtgattaaaataaaatataatttaggtgtacatcaaataaaaaccttaaagtttagaaaggcaccgaataattttgcatagaagatattagtaaatttataaaaataaaagaaatgtagttgtcaagttgtcttcttttttttggataaaaatagcagttggcttatgtcattcttttacaacctccatgccacttgtccaattgttgacacttaactaattagtttgattcatgtatgaatactaaataattttttaggactgactcaaatatttttatattatcatagtaatatttatctaatttttaggaccacttattactaaataataaattaactacaactatattattgttgtgaaacaacaacgttttggttgttatgatgaaacgtacactatatcagtatgaaaaattcaaaacgattagtataaattatattgaaaatttgatatttttctattcttaatcagacgtattgggtttcatattttaaaaagggactaaacttagaagagaagtttgtttgaaactacttttgtctctttcttgttcccatttctctcttagatttcaaaaagtgaactactttatctccttctttgttcacattttattttattctattataaatatggcatcctcatattgagatttttagaaattattctaatcattcacagtgcaaaagaagaatggaatctcctgctactaaattacctgcacctctgctgatgttatcttcttctccattccttctcccttctcctaataagagctcctccatcttccttccacgtaaattagggccgctacctccaaaatattattattacaattgctgccatcctaagagtagatcaatctcagtagtatcaatggcaaataaggaggaggcagagacaagtaagaagaagcccaaaccattaaaagtactaattaccaaagtggatccgaagccgaggaagggcatggcatccgtcgcagtggacttactcgagaaggcctttgtatacctattgtccggaaattctgcagctgatcgtagtagtagtagtggtcgtcgtcgtcgtaaagagcattactacctctccggcaattatgcgcccgtcggacacgaaaccccgccctccgaccacctccccattcatggatcccttcctgaatgcttgaatggagtgtttctgagagttggtcctaaccccaagtttgctcccgtagccggatacaattgggtcgatggagatggaatgattcatggattgcgtattaaagatggaaaagcaacttatctatctcgatatattaaaacgtcacggtttaaacaagaagaatattttggaagagcaaaatttatgaagattggagatctaaggggattgcttgggttctttacgatcttaatactagtacttcgaacaacattgaaagtaatagacatttcatatggaagagggacgggtaatacagctcttgtgtatcataatggcttactattggctctatcagaagaagataaaccttatgttgttaaagttttagaagatggagacttgcaaactcttgggatattggattatgacaagaaattgtcacatccattcaccgctcatccaaagatcgatccgttaactgatgagatgtttacctttggatattccatctcgcctccgtatcttacttatcgagtcatttccaaggatggagtgatgcaagatccagtgcaaatctcaattacatcccctaccataatgcatgattttgctattactgaaaattatgccatcttcatggacctgcccttgtatttccaaccagaggaaatggtaaaggggaaatttgtctcttcatttcaccctacaaaaagagctcgtatcggtgtgcttccacgatatgcaaaagacgagcatccaattcgatggttcgatcttccaagttgcttcatgactcataatgcaaatgcttgggaagagaatgatgaagttgtgctattcacatgtcgccttgagagtcctgatcttgacatgcttagtggacctgcggaagaagagattgggaattcaaaaagtgagctttacgaaatgaggttcaatttgaaaactggaattacttcacaaaagcaactatctgtacctagtgttgattttcctcggatcaaccaaagttatactggcaggaaacagcaatatgtttattgtactcttggcaacaccaagattaagggcattgtgaagtttgatctgcaaattgaaccagaagccggaaagacaatgcttgaagttggaggaaatgtacaaggcatctttgagttgggacctagaagatatggttcagaggcaatatttgtgccatgccaacctggcatcaaatctgatgaggatgacggttacttgatattctttgtacacgacgaaaacaatgggaaatctgaggtcaatgtcatcgatgcaaagacaatgtctgcagaacctgtggctgttgtggaacttccaagcagggttccatatggattccatgccttgtttctgaatgaggaagaacttcagaagcaccaagcagagacatgagcttcggccatgctagagtccgcaaaaatcaccagtctctctctacaaatctatctctctctatttttctccagaataatgtgtgagtagttcccagataagggaattagggttcttatagggtttcgctcatgtgttgagcatataagaaacccttagtatgtatttgtatttgtaaaatacttctatcaataaaatttctaattcctaaaaccaaaatccagtgacctcgctgtcatgagacgaattctgacaggatatattggcgggtaaacctaagagaaaagagcgtttattagaataatcggatatttaaaagggcgtgaaaaggtttatccgttcgtccatttgtatgtgcatgccaaccacagggttcccctcgggatcaaagtactttgatccaacccctccgctgctatagtgcagtcggcttctgacgttcagtgcagccgtcatctgaaaacgacatgtcgcacaagtcctaagttacgcgacaggctgccgccctgcccttttcctggcgttttcttgtcgcgtgttttagtcgcataaagtagaatacttgcgactagaaccggagacattacgccatgaacaagagcgccgccgctggcctgctgggctatgcccgcgtcagcaccgacgaccaggacttgaccaaccaacgggccgaactgcacgcggccggctgcaccaagctgttttccgagaagatcaccggcaccaggcgcgaccgcccggagctggccaggatgcttgaccacctacgccctggcgacgttgtgacagtgaccaggctagaccgcctggcccgcagcacccgcgacctactggacattgccgagcgcatccaggaggccggcgcgggcctgcgtagcctggcagagccgtgggccgacaccaccacgccggccggccgcatggtgttgaccgtgttcgccggcattgccgagttcgagcgttccctaatcatcgaccgcacccggagcgggcgcgaggccgccaaggcccgaggcgtgaagtttggcccccgccctaccctcaccccggcacagatcgcgcacgcccgcgagctgatcgaccaggaaggccgcaccgtgaaagaggcggctgcactgcttggcgtgcatcgctcgaccctgtaccgcgcacttgagcgcagcgaggaagtgacgcccaccgaggccaggcggcgcggtgccttccgtgaggacgcattgaccgaggccgacgccctggcggccgccgagaatgaacgccaagaggaacaagcatgaaaccgcaccaggacggccaggacgaaccgtttttcattaccgaagagatcgaggcggagatgatcgcggccgggtacgtgttcgagccgcccgcgcacctctcaaccgtgcggctgcatgaaatcctggccggtttgtctgatgccaagctggcggcctggccggccagcttggccgctgaagaaaccgagcgccgccgtctaaaaaggtgatgtgtatttgagtaaaacagcttgcgtcatgcggtcgctgcgtatatgatccgatgagtaaataaacaaatacgcaaggggaacgcatgaaggttatcgctgtacttaaccagaaaggcgggtcaggcaagacgaccatcggaacccatctagcccgcgccctgcaactcgccggggccgatgttctgttagtcgattccgatccccagggcagtgcccgcgattgggcggccgtgcgggaagatcaaccgctaaccgttgtcggcatcgaccgcccgacgattgaccgcgacgtgaaggccatcggccggcgcgacttcgtagtgatcgacggagcgccccaggcggcggacttggctgtgtccgcgatcaaggcagccgacttcgtgctgattccggtgcagccaagcccttacgacatatgggccaccgccgacctggtggagctggttaagcagcgcattgaggtcacggatggaaggctacaagcggcctttgtcgtgtcgcgggcgatcaaaggcacgcgcatcggcggtgaggttgccgaggcgctggccgggtacgagctgcccattcttgagtcccgtatcacgcagcgcgtgagctacccaggcactgccgccgccggcacaaccgttcttgaatcagaacccgagggcgacgctgcccgcgaggtccaggcgctggccgctgaaattaaatcaaaactcatttgagttaatgaggtaaagagaaaatgagcaaaagcacaaacacgctaagtgccggccgtccgagcgcacgcagcagcaaggctgcaacgttggccagcctggcagacacgccagccatgaagcgggtcaactttcagttgccggcggaggatcacaccaagctgaagatgtacgcggtacgccaaggcaagaccattaccgagctgctatctgaatagatcgcgcagctaccagagtaaatgagcaaatgaataaatgagtagatgaattttagcggctaaaggaggcggcatggaaaatcaagaacaaccaggcaccgacgccgtggaatgccccatgtgtggaggaacgggcggttggccaggcgtaagcggctgggttgtctgccggccctgcaatggcactggaacccccaagcccgaggaatcggcgtgacggtcgcaaaccatccggcccggtacaaatcggcgcggcgctgggtgatgacctggtggagaagttgaaggccgcgcaggccgcccagcggcaacgcatcgaggcagaagcacgccccggtgaatcgtggcaagcggccgctgatcgaatccgcaaagaatcccggcaaccgccggcagccggtgcgccgtcgattaggaagccgcccaagggcgacgagcaaccagattttttcgttccgatgctctatgacgtgggcacccgcgatagtcgcagcatcatggacgtggccgttttccgtctgtcgaagcgtgaccgacgagctggcgaggtgatccgctacgagcttccagacgggcacgtagaggtttccgcagggccggccggcatggccagtgtgtgggattacgacctggtactgatggcggtttcccatctaaccgaatccatgaaccgataccgggaagggaagggagacaagcccggccgcgtgttccgtccacacgttgcggacgtactcaagttctgccggcgagccgatggcggaaagcagaaagacgacctggtagaaacctgcattcggttaaacaccacgcacgttgccatgcagcgtacgaagaaggccaagaacggccgcctggtgacggtatccgagggtgaagccttgattagccgctacaagatcgtaaagagcgaaaccgggcggccggagtacatcgagatcgagctagctgattggatgtaccgcgagatcacagaaggcaagaacccggacgtgctgacggttcaccccgattactttttgatcgatcccggcatcggccgttttctctaccgcctggcacgccgcgccgcaggcaaggcagaagccagatggttgttcaagacgatctacgaacgcagtggcagcgccggagagttcaagaagttctgtttcaccgtgcgcaagctgatcgggtcaaatgacctgccggagtacgatttgaaggaggaggcggggcaggctggcccgatcctagtcatgcgctaccgcaacctgatcgagggcgaagcatccgccggttcctaatgtacggagcagatgctagggcaaattgccctagcaggggaaaaaggtcgaaaaggactctttcctgtggatagcacgtacattgggaacccaaagccgtacattgggaaccggaacccgtacattgggaacccaaagccgtacattgggaaccggtcacacatgtaagtgactgatataaaagagaaaaaaggcgatttttccgcctaaaactctttaaaacttattaaaactcttaaaacccgcctggcctgtgcataactgtctggccagcgcacagccgaagagctgcaaaaagcgcctacccttcggtcgctgcgctccctacgccccgccgcttcgcgtcggcctatcgcggccgctggccgctcaaaaatggctggcctacggccaggcaatctaccagggcgcggacaagccgcgccgtcgccactcgaccgccggcgcccacatcaaggcaccctgcctcgcgcgtttcggtgatgacggtgaaaacctctgacacatgcagctcccggtgacggtcacagcttgtctgtaagcggatgccgggagcagacaagcccgtcagggcgcgtcagcgggtgttggcgggtgtcggggcgcagccatgacccagtcacgtagcgatagcggagtgtatactggcttaactatgcggcatcagagcagattgtactgagagtgcaccatatgcggtgtgaaataccgcacagatgcgtaaggagaaaataccgcatcaggcgctcttccgcttcctcgctcactgactcgctgcgctcggtcgttcggctgcggcgagcggtatcagctcactcaaaggcggtaatacggttatccacagaatcaggggataacgcaggaaagaacatgtgagcaaaaggccagcaaaaggccaggaaccgtaaaaaggccgcgttgctggcgtttttccataggctccgcccccctgacgagcatcacaaaaatcgacgctcaagtcagaggtggcgaaacccgacaggactataaagataccaggcgtttccccctggaagctccctcgtgcgctctcctgttccgaccctgccgcttaccggatacctgtccgcctttctcccttcgggaagcgtggcgctttctcatagctcacgctgtaggtatctcagttcggtgtaggtcgttcgctccaagctgggctgtgtgcacgaaccccccgttcagcccgaccgctgcgccttatccggtaactatcgtcttgagtccaacccggtaagacacgacttatcgccactggcagcagccactggtaacaggattagcagagcgaggtatgtaggcggtgctacagagttcttgaagtggtggcctaactacggctacactagaaggacagtatttggtatctgcgctctgctgaagccagttaccttcggaaaaagagttggtagctcttgatccggcaaacaaaccaccgctggtagcggtggtttttttgtttgcaagcagcagattacgcgcagaaaaaaaggatctcaagaagatcctttgatcttttctacggggtctgacgctcagtggaacgaaaactcacgttaagggattttggtcatgcattctaggtgattagaaaaactcatcgagcatcaaatgaaactgcaatttattcatatcaggattatcaataccatatttttgaaaaagccgtttctgtaatgaaggagaaaactcaccgaggcagttccataggatggcaagatcctggtatcggtctgcgattccgactcgtccaacatcaatacaacctattaatttcccctcgtcaaaaataaggttatcaagtgagaaatcaccatgagtgacgactgaatccggtgagaatggcaaaagtttatgcatttctttccagacttgttcaacaggccagccattacgctcgtcatcaaaatcactcgcatcaaccaaaccgttattcattcgtgattgcgcctgagcgagtcgaaatacgcgatcgctgttaaaaggacaattacaaacaggaatcgaatgcaaccggcgcaggaacactgccagcgcatcaacaatattttcacctgaatcaggatattcttctaatacctggaatgctgttttccctgggatcgcagtggtgagtaaccatgcatcatcaggagtacggataaaatgcttgatggtcggaagaggcataaattccgtcagccagtttagtctgaccatctcatctgtaacatcattggcaacgctacctttgccatgtttcagaaacaactctggcgcatcgggcttcccatacaatcggtagattgtcgcacctgattgcccgacattatcgcgagcccatttatacccatataaatcagcatccatgttggaatttaatcgcggccttgagcaagacgtttcccgttgaatatggctcataacagaacttattatttccttcctcttttctacagtatttaaagataccccaagaagctaattataacaagacgaactccaattcactgttccttgcattctaaaaccttaaataccagaaaacagctttttcaaagttgttttcaaagttggcgtataacatagtatcgacggagccgattttgaaaccgcggtgatcacaggcagcaacgctctgtcatcgttacaatcaacatgctaccctccgcgagatcatccgtgtttcaaacccggcagcttagttgccgttcttccgaatagcatcggtaacatgagcaaagtctgccgccttacaacggctctcccgctgacgccgtcccggactgatgggctgcctgtatcgagtggtgattttgtgccgagctgccggtcggggagctgttggctggctggtggcaggatatattgtggtgtaaacataacgaattcgtctca

SEQ ID NO: 23 - DNA, 16761 bp, synthetic construct
  source 1..16761: mol_type = other DNA; plasmid = DNA contruct O3 = pDGB3alpha1[p35S:UGT2:T35S-p35S:UGT709G1:T35S-p35S:CCD2L:T35S-pNos:Hyg:T35S]
ggagactagagccaagctgatctcctttgccccggagatcaccatggacgactttctctatctctacgatctaggaagaaagttcgacggagaaggtgacgataccatgttcaccaccgataatgagaagattagcctcttcaatttcagaaagaatgctgacccacagatggttagagaggcctacgcggcaggtctgatcaagacgatctacccgagtaataatctccaggagatcaaataccttcccaagaaggttaaagatgcagtcaaaagattcaggactaactgcatcaagaacacagagaaagatatatttctcaagatcagaagtactattccagtatggacgattcaaggcttgcttcataaaccaaggcaagtaatagagattggagtctctaagaaagtagttcctactgaatcaaaggccatggagtcaaaaattcagatcgaggatctaacagaactcgccgtgaagactggcgaacagttcatacagagtcttttacgactcaatgacaagaagaaaatcttcgtcaacatggtggagcacgacactctcgtctactccaagaatatcaaagatacagtctcagaagaccaaagggctattgagacttttcaacaaagggtaatatcgggaaacctcctcggattccattgcccagctatctgtcacttcatcaaaaggacagtagaaaaggaaggtggcacctacaaatgccatcattgcgataaaggaaaggctatcgttcaagatgcctctgccgacagtggtcccaaagatggacccccacccacgaggagcatcgtggaaaaagaagacgttccaaccacgtcttcaaagcaagtggattgatgtgatatctccactgacgtaagggatgacgcacaatcccactatccttcgcaagacccttcctctatataaggaagttcatttcatttggagaggactccggtatttttacaacaataccacaacaaaacaaacaacaaacaacattacaatttactattctagtcgaaatgttgaacggcaacaaatgccacatcctcctcctcccctgtccagcacaaggccatatcaaccccattctccaattcggcaagcgactggcctctcacaacctcctcaccacactcgtcaacacccggttcctctccaactcgaccaaatccgaacccggtccggtcaacatccagtgcatatccgacggattcgatcccggtgggatgaatgcagcacctagtcgtcgggcctatttcgaccgacctcagagtcggtcgggtcagaaacatgttggcctcatcgagtcactccggtccagaggccgacccggcgcatgttttggtctacgacccgttcccctctgggcaatgaacgtagccgagcggtccgggctgcggtcggtcgcattctttactcagccgtgtgcagtggacacaatctaccgccacgtgtgggagggacgaattaaggttccggttgccgagccggtccggttgcctggattgcccccactcgagcctagtgatctgccgtgcgttcgtaacggattcggacgagtcgttaacccggatctcttgccacttcgagtgaatcagcacaaaaatttggacaaagctgacatgatggggaggaactccatatacgagctagaggcggatttgttggatgggtcccgattaccattaccggtgaagtcgattgggccgaccgtgccgtctacttatctcgacaaccgaatcccgtcggattcacactatggattcaatctatacacccctgacactactccctacttggactggctcgactccaaggccccgaactctgtcatctatgtctcatttggtagtttgtccagtctgagccctgatcaaaccaatgagattgcgtcgggtctgatcgccaccaacaaaagctttatttgggtggtacgcacttcggagttagccaaactccctgccaacttcacccaagagaatgcgagccgtgggctggttgtgacctggtgcgaccaactcgatctcctcgcacacgttgcgaccggttgcttcgtgactcactgcggatggaactcgactatggaaggtgtcgcacttggtgtgccgatggtgggagtgccgcagtggtcggaccagcctatgaatgccaagtatgtagaggatgtgtggaaggtcggcgtgagggcgaagacttatgggaaggattttgtgagaggggaggagttcaaaagatgtgtggaggaggtgatggatggagagaggagtggaaagattagagagaatgccgcaaggtggtgtaagttggccaaggactctgttagtgagggtgggagttctgacaagtgtatcaaggagttcatacatcagtgttgcaatgactccaaaatttccttagtttaagcttcggccatgctagagtccgcaaaaatcaccagtctctctctacaaatctatctctctctatttttctccagaataatgtgtgagtagttcccagataagggaattagggttcttatagggtttcgctcatgtgttgagcatataagaaacccttagtatgtatttgtatttgtaaaatacttctatcaataaaatttctaattcctaaaaccaaaatccagtgacctcgctgtcaggagactagagccaagctgatctcctttgccccggagatcaccatggacgactttctctatctctacgatctaggaagaaagttcgacggagaaggtgacgataccatgttcaccaccgataatgagaagattagcctcttcaatttcagaaagaatgctgacccacagatggttagagaggcctacgcggcaggtctgatcaagacgatctacccgagtaataatctccaggagatcaaataccttcccaagaaggttaaagatgcagtcaaaagattcaggactaactgcatcaagaacacagagaaagatatatttctcaagatcagaagtactattccagtatggacgattcaaggcttgcttcataaaccaaggcaagtaatagagattggagtctctaagaaagtagttcctactgaatcaaaggccatggagtcaaaaattcagatcgaggatctaacagaactcgccgtgaagactggcgaacagttcatacagagtcttttacgactcaatgacaagaagaaaatcttcgtcaacatggtggagcacgacactctcgtctactccaagaatatcaaagatacagtctcagaagaccaaagggctattgagacttttcaacaaagggtaatatcgggaaacctcctcggattccattgcccagctatctgtcacttcatcaaaaggacagtagaaaaggaaggtggcacctacaaatgccatcattgcgataaaggaaaggctatcgttcaagatgcctctgccgacagtggtcccaaagatggacccccacccacgaggagcatcgtggaaaaagaagacgttccaaccacgtcttcaaagcaagtggattgatgtgatatctccactgacgtaagggatgacgcacaatcccactatccttcgcaagacccttcctctatataaggaagttcatttcatttggagaggactccggtatttttacaacaataccacaacaaaacaaacaacaaacaacattacaatttactattctagtcgaaatggctgagaaagaagcaaatacccatgtcgtcctcttccccttgccaggccaagggcacatcggctcaatgttgaaactggcacagcttctttccaccgccggattctacgtcactttcgtccacaccgaacgcaactaccgtcgctacctcctcacctccacgtccttccacgtccccaagttccggttccgcaccatccccgacggttttcccgacgacgattcccgctcgcccctcccttttctcgagctccaagagtcgctggacacgaaatgtcgggggcattatcgggaattgttggtcgctgtcgacgaccaagaagagtggcccccagtcacttgtgtcgtggctgatcaagctcttccactctcactcgaagttcccgacgagttggggattcctgtaatgatactcgcaccacacagtgcgtgcagtatattgacgagttattcgattccggagcttataaggggaggtgaactccctatcccagatggggccaatatggatgaactattacaaggcgtactgggattggaaggtatcgtgaggcgtagggatatgtccatcagaagcgccaagtccatccaagatccatttcttcaattcgaagtgaaaatgagcaaaaacttgcccagaggaagagctctcatcctgaacactacagaatcgatagactctctttctttgcgacacattcggtcgatctgtcccactacctacgcactcgggcccttccacgtccttctcaggaacataaaagacgagtcccactccgcaagcctttccgaagaggacaggtcctgcatcgcctggctggactcgaaaccgaacaagtccgcggtctacgtgagtttcggtagcctcgccgccatggcgagagaagcatttcttgagtttcagcagggattgctcgacagcgggtattacttcttgtgggtgatccggcccgatatggtggaaggggggctggaagagagcgagctgaccgcgagcgaacaacgctactttgtgaagtgggccccacaggaggaggttcttgcgcacccggcggtagggtgtttcttgacgcacagcggttggaactctacgttggagagtatctttgcgggagtgccgatgatatgttggcctttctttgcggaccagctgattaacagtaggtttgcgagcgaggtgtggaaaattgccttggatatgaaggatttgtgcggaaggagccacgtggagaggatggtgaaggaagttatgagtggagagaaaggcgaagagctaaggaattctagctgcgagatggcagatagggtgaagaagagtgcagaggaaggtggctcttcctacgccaacttcaaagagttggttggacatatcaaatctttgagcttaccagcagaaagaggagaaaatggtggtgaaggaatgagtgtacaagcgccgagtaaacttttcctcctcaacgctgaggacggaaaacatgtccttaaaagtgacgaaccgtcggaacaaaggggtccacaatttaatccaaattttcttcggacctgagcttcggccatgctagagtccgcaaaaatcaccagtctctctctacaaatctatctctctctatttttctccagaataatgtgtgagtagttcccagataagggaattagggttcttatagggtttcgctcatgtgttgagcatataagaaacccttagtatgtatttgtatttgtaaaatacttctatcaataaaatttctaattcctaaaaccaaaatccagtgacctcgctgtcaggagagcgcgagtcggtcccattattgaagcatttatcagggttattgtctcatgagcggatacatatttgaatgtatttagaaaaataaacaaataggggttccgcgcacatttccccgaaaagtgccacctgacgtctaagaaaccattattatcatgacattaacctataaaaataggcgtatcacgaggccctttcgtcttcaagaattagcttggcaattcccgatctagtaacatagatgacaccghgcgcgataatttatcctagtttgcgcgctatattttgttttctatcgcgtattaaatgtataattgcgggactctaatcataaaaacccatctcataaataacgtcatgcattacatgttaattattacatgcttaacgtaattcaacagaaattatatgataatcgtcgcaagaccggcaacaggattcaatcttaagaaactttattgccaaatgtttgaacgatcgggatcgaagatccattccaagctcattcctttgccctcggacgagtgctggggcgtcggtttccactatcggcgagtacttctacacagccatcggtccagacggccgcgcttctgcgggcgatttgtgtacgcccgacagtcccggctccggatcggacgattgcgtcgcatcgaccctgcgcccaagctgcatcatcgaaattgccgtcaaccaagctctgatagagttggtcaagaccaatgcggagcatatacgcccggagtcgtggcgatcctgcaagctccggatgcctccgctcgaagtagcgcgtctgctgctccatacaagccaaccacggcctccagaagaagatgttggcgacctcgtattgggaatccccgaacattgcctcgctccagtcaatgaccgctgttatgcggccattgtccgtcaggacattgttggagccgaaatccgcgtgcacgaggtgccggacttcggggcagtcctcggcccaaagcatcagctcatcgagagcctgcgcgacggacgcactgacggtgtcgtccatcacagtttgccagtgatacacatggggatcagcaatcgcgcatatgaaatcacgccatgtagtgtattgaccgattccttgcggtccgaatgggccgaacccgctcgtctggctaagatcggccgcagcgatcgcatccatggcctccgcgaccggctgcagaacagcgggcagttcggtttcaggcaggtcttgcaacgtgacaccctgtgcacggcgggagatgcaataggtcaggctctcgctgaattccccaatgtcaagcacttccggaatcgggagcgcggccgatgcaaagtgccgataaacataacgatctttgtagaaaccatcggcgcagctatttacccgcaggacatatccacgccctcctacatcgaagctgaaagcacgagattcttcgccctccgagagctgcatcaggtcggacacgctgtcgaacttttcgatcagaaacttctcgacagacgtcgcggtgagttcaggctttttcattgcctcgatcgagttgagagtgaatatgagactctaattggataccgaggggaatttatggaacgtcagtggagcatttttgacaagaaatatttgctagctgatagtgaccttaggcgacttttgaacgcgcaataatggtttctgacgtatgtgcttagctcattaaactccagaaacccgcggctcagtggctccttcaacgttgcggttctgtcagttccaaacgtaaaacggcttgtcccgcgtcatcggcgggggtcataccgtgactcccttaattctcatgtatctccgtcaggagactagagccaagctgatctcctttgccccggagatcaccatggacgactttctctatctctacgatctaggaagaaagttcgacggagaaggtgacgataccatgttcaccaccgataatgagaagattagcctcttcaatttcagaaagaatgctgacccacagatggttagagaggcctacgcggcaggtctgatcaagacgatctacccgagtaataatctccaggagatcaaataccttcccaagaaggttaaagatgcagtcaaaagattcaggactaactgcatcaagaacacagagaaagatatatttctcaagatcagaagtactattccagtatggacgattcaaggcttgcttcataaaccaaggcaagtaatagagattggagtctctaagaaagtagttcctactgaatcaaaggccatggagtcaaaaattcagatcgaggatctaacagaactcgccgtgaagactggcgaacagttcatacagagtcttttacgactcaatgacaagaagaaaatcttcgtcaacatggtggagcacgacactctcgtctactccaagaatatcaaagatacagtctcagaagaccaaagggctattgagacttttcaacaaagggtaatatcgggaaacctcctcggattccattgcccagctatctgtcacttcatcaaaaggacagtagaaaaggaaggtggcacctacaaatgccatcattgcgataaaggaaaggctatcgttcaagatgcctctgccgacagtggtcccaaagatggacccccacccacgaggagcatcgtggaaaaagaagacgttccaaccacgtcttcaaagcaagtggattgatgtgatatctccactgacgtaagggatgacgcacaatcccactatccttcgcaagacccttcctctatataaggaagttcatttcatttggagaggactccggtatttttacaacaataccacaacaaaacaaacaacaaacaacattacaatttactattctagtcgaaatgcatggaatctcctactactaaattacctgcacctctgctgatgttatcttcttctccactccttctcccttctccttataagagctcctccatcttccttccacgtaaatttgggccgctacctcctaattattattacaattgctgccatcctaagagtagaccaatctcagtagtatcaatggcaaataaggaggaggcagagaagaggaagaagaagcccaaaccattaaaagtactaattaccaaagtggacccgaagccgaggaagggcatggcatccgtcgcagtggacttactcgagaaggcctttgtatacctattgtacggaaattctgcagctgatcgtagtagtggtcgtcgtcgtcgtaaagagcattactacctctccggcaattatgcgcccgtcggacacgaaaccccaccctccgaccacctccccgttcatggatcccttcctgaatgcttgaatggagtgtttctgagagttggccctaaccccaagtttgctcccgtagccggatacaattgggtcgatggagatggaatgattcatggattgcgtattaaagatggaaaagcaacttatctatcccgatatattaaaacgtcacggtttaaacaagaagaatattttggaagagcaaaatttatgaagattggagatctaagaggattgcttggattctttacgatcttaatactagtacttcgaacaacattgaaagtaatagacatttcatatggaagggggacaggtaatacagctcttgtatatcataatggcttactattggctctatcagaagaagataaaccttatgttgttaaagttttagaagatggagacttgcaaactcttgggatattggattatgacaagaaattgtcacatccattcaccgctcatccaaagatcgatccgttaaccgatgagatgtttacctttggatattccctctcgcctccgtatcttacttatcgagtcatttccaaggatggagtgatgcaagatccagtgcaaatctcaattacatcccctaccataatgcatgattttgctattactgaaaattatgccatcttcatggacctgcccttgtatttccaaccagaggaaatggtaaaggggaaatttgtctcttcatttcaccccacaaaaagagctcgtatcggtgtgcttccacgatatgcagaagacgagcatccaattcgatggtttgatcttccaagttgcttcatgactcataatgcaaatgcttgggaagagaatgatgaagttgtgctattcacatgtcgccttgagagtcctgatcttgacatgcttagtggacctgcggaagaagagattgggaattcaaaaagtgagctttatgaaatgaggttcaatttgaaaactggaattacttcacaaaagcaactatctgtacctagtgttgattttcctcggatcaaccaaagttatactggcaggaaacagcaatatgtttattgtactcttggcaacaccaagattaagggcattgtgaagtttgatctgcaaattgaaccagaagccggaaagacaatgcttgaagttggaggaaatgtacaaggcatctttgagttgggacctagaagatatggttcagaggcaatatttgtgccatgccaacctggcatcaaatctgatgaggatgacggttacttgatattctttgtacacgacgaaaacaatgggaaatctgaggtcaatgtcatcgatgcaaagacaatgtctgcagaacctgtggctgttgtgcaacttccaagcagggttccatatggattccatgccttgtttgagcttcggccatgctagagtccgcaaaaatcaccagtctctctctacaaatctatctctctctatttttctccagaataatgtgtgagtagttcccagataagggaattagggttcttatagggtttcgctcatgtgttgagcatataagaaacccttagtatgtatttgtatttgtaaaatacttctatcaataaaatttctaattcctaaaaccaaaatccagtgacctcgctgtcatgagacgaattctgacaggatatattggcgggtaaacctaagagaaaagagcgtttattagaataatcggatatttaaaagggcgtgaaaaggtttatccgttcgtccatttgtatgtgcatgccaaccacagggttcccctcgggatcaaagtactttgatccaacccctccgctgctatagtgcagtcggcttctgacgttcagtgcagccgtcatctgaaaacgacatgtcgcacaagtcctaagttacgcgacaggctgccgccctgcccttttcctggcgttttcttgtcgcgtgttttagtcgcataaagtagaatacttgcgactagaaccggagacattacgccatgaacaagagcgccgccgctggcctgctgggctatgcccgcgtcagcaccgacgaccaggacttgaccaaccaacgggccgaactgcacgcggccggctgcaccaagctgttttccgagaagatcaccggcaccaggcgcgaccgcccggagctggccaggatgcttgaccacctacgccctggcgacgttgtgacagtgaccaggctagaccgcctggcccgcagcacccgcgacctactggacattgccgagcgcatccaggaggccggcgcgggcctgcgtagcctggcagagccgtgggccgacaccaccacgccggccggccgcatggtgttgaccgtgttcgccggcattgccgagttcgagcgttccctaatcatcgaccgcacccggagcgggcgcgaggccgccaaggcccgaggcgtgaagtttggcccccgccctaccctcaccccggcacagatcgcgcacgcccgcgagctgatcgaccaggaaggccgcaccgtgaaagaggcggctgcactgcttggcgtgcatcgctcgaccctgtaccgcgcacttgagcgcagcgaggaagtgacgcccaccgaggccaggcggcgcggtgccttccgtgaggacgcattgaccgaggccgacgccctggcggccgccgagaatgaacgccaagaggaacaagcatgaaaccgcaccaggacggccaggacgaaccgtttttcattaccgaagagatcgaggcggagatgatcgcggccgggtacgtgttcgagccgcccgcgcacctctcaaccgtgcggctgcatgaaatcctggccggtttgtctgatgccaagctggcggcctggccggccagcttggccgctgaagaaaccgagcgccgccgtctaaaaaggtgatgtgtatttgagtaaaacagcttgcgtcatgcggtcgctgcgtatatgatccgatgagtaaataaacaaatacgcaaggggaacgcatgaaggttatcgctgtacttaaccagaaaggcgggtcaggcaagacgaccatcggaacccatctagcccgcgccctgcaactcgccggggccgatgttctgttagtcgattccgatccccagggcagtgcccgcgattgggcggccgtgcgggaagatcaaccgctaaccgttgtcggcatcgaccgcccgacgattgaccgcgacgtgaaggccatcggccggcgcgacttcgtagtgatcgacggagcgccccaggcggcggacttggctgtgtccgcgatcaaggcagccgacttcgtgctgattccggtgcagccaagcccttacgacatatgggccaccgccgacctggtggagctggttaagcagcgcattgaggtcacggatggaaggctacaagcggcctttgtcgtgtcgcgggcgatcaaaggcacgcgcatcggcggtgaggttgccgaggcgctggccgggtacgagctgcccattcttgagtcccgtatcacgcagcgcgtgagctacccaggcactgccgccgccggcacaaccgttcttgaatcagaacccgagggcgacgctgcccgcgaggtccaggcgctggccgctgaaattaaatcaaaactcatttgagttaatgaggtaaagagaaaatgagcaaaagcacaaacacgctaagtgccggccgtccgagcgcacgcagcagcaaggctgcaacgttggccagcctggcagacacgccagccatgaagcgggtcaactttcagttgccggcggaggatcacaccaagctgaagatgtacgcggtacgccaaggcaagaccattaccgagctgctatctgaatagatcgcgcagctaccagagtaaatgagcaaatgaataaatgagtagatgaattttagcggctaaaggaggcggcatggaaaatcaagaacaaccaggcaccgacgccgtggaatgccccatgtgtggaggaacgggcggttggccaggcgtaagcggctgggttgtctgccggccctgcaatggcactggaacccccaagcccgaggaatcggcgtgacggtcgcaaaccatccggcccggtacaaatcggcgcggcgctgggtgatgacctggtggagaagttgaaggccgcgcaggccgcccagcggcaacgcatcgaggcagaagcacgccccggtgaatcgtggcaagcggccgctgatcgaatccgcaaagaatcccggcaaccgccggcagccggtgcgccgtcgattaggaagccgcccaagggcgacgagcaaccagattttttcgttccgatgctctatgacgtgggcacccgcgatagtcgcagcatcatggacgtggccgttttccgtctgtcgaagcgtgaccgacgagctggcgaggtgatccgctacgagcttccagacgggcacgtagaggtttccgcagggccggccggcatggccagtgtgtgggattacgacctggtactgatggcggtttcccatctaaccgaatccatgaaccgataccgggaagggaagggagacaagcccggccgcgtgttccgtccacacgttgcggacgtactcaagttctgccggcgagccgatggcggaaagcagaaagacgacctggtagaaacctgcattcggttaaacaccacgcacgttgccatgcagcgtacgaagaaggccaagaacggccgcctggtgacggtatccgagggtgaagccttgattagccgctacaagatcgtaaagagcgaaaccgggcggccggagtacatcgagatcgagctagctgattggatgtaccgcgagatcacagaaggcaagaacccggacgtgctgacggttcaccccgattactttttgatcgatcccggcatcggccgttttctctaccgcctggcacgccgcgccgcaggcaaggcagaagccagatggttgttcaagacgatctacgaacgcagtggcagcgccggagagttcaagaagttctgtttcaccgtgcgcaagctgatcgggtcaaatgacctgccggagtacgatttgaaggaggaggcggggcaggctggcccgatcctagtcatgcgctaccgcaacctgatcgagggcgaagcatccgccggttcctaatgtacggagcagatgctagggcaaattgccctagcaggggaaaaaggtcgaaaaggactctttcctgtggatagcacgtacattgggaacccaaagccgtacattgggaaccggaacccgtacattgggaacccaaagccgtacattgggaaccggtcacacatgtaagtgactgatataaaagagaaaaaaggcgatttttccgcctaaaactctttaaaacttattaaaactcttaaaacccgcctggcctgtgcataactgtctggccagcgcacagccgaagagctgcaaaaagcgcctacccttcggtcgctgcgctccctacgccccgccgcttcgcgtcggcctatcgcggccgctggccgctcaaaaatggctggcctacggccaggcaatctaccagggcgcggacaagccgcgccgtcgccactcgaccgccggcgcccacatcaaggcaccctgcctcgcgcgtttcggtgatgacggtgaaaacctctgacacatgcagctcccggtgacggtcacagcttgtctgtaagcggatgccgggagcagacaagcccgtcagggcgcgtcagcgggtgttggcgggtgtcggggcgcagccatgacccagtcacgtagcgatagcggagtgtatactggcttaactatgcggcatcagagcagattgtactgagagtgcaccatatgcggtgtgaaataccgcacagatgcgtaaggagaaaataccgcatcaggcgctcttccgcttcctcgctcactgactcgctgcgctcggtcgttcggctgcggcgagcggtatcagctcactcaaaggcggtaatacggttatccacagaatcaggggataacgcaggaaagaacatgtgagcaaaaggccagcaaaaggccaggaaccgtaaaaaggccgcgttgctggcgtttttccataggctccgcccccctgacgagcatcacaaaaatcgacgctcaagtcagaggtggcgaaacccgacaggactataaagataccaggcgtttccccctggaagctccctcgtgcgctctcctgttccgaccctgccgcttaccggatacctgtccgcctttctcccttcgggaagcgtggcgctttctcatagctcacgctgtaggtatctcagttcggtgtaggtcgttcgctccaagctgggctgtgtgcacgaaccccccgttcagcccgaccgctgcgccttatccggtaactatcgtcttgagtccaacccggtaagacacgacttatcgccactggcagcagccactggtaacaggattagcagagcgaggtatgtaggcggtgctacagagttcttgaagtggtggcctaactacggctacactagaaggacagtatttggtatctgcgctctgctgaagccagttaccttcggaaaaagagttggtagctcttgatccggcaaacaaaccaccgctggtagcggtggtttttttgtttgcaagcagcagattacgcgcagaaaaaaaggatctcaagaagatcctttgatcttttctacggggtctgacgctcagtggaacgaaaactcacgttaagggattttggtcatgcattctaggtgattagaaaaactcatcgagcatcaaatgaaactgcaatttattcatatcaggattatcaataccatatttttgaaaaagccgtttctgtaatgaaggagaaaactcaccgaggcagttccataggatggcaagatcctggtatcggtctgcgattccgactcgtccaacatcaatacaacctattaatttcccctcgtcaaaaataaggttatcaagtgagaaatcaccatgagtgacgactgaatccggtgagaatggcaaaagtttatgcatttctttccagacttgttcaacaggccagccattacgctcgtcatcaaaatcactcgcatcaaccaaaccgttattcattcgtgattgcgcctgagcgagtcgaaatacgcgatcgctgttaaaaggacaattacaaacaggaatcgaatgcaaccggcgcaggaacactgccagcgcatcaacaatattttcacctgaatcaggatattcttctaatacctggaatgctgttttccctgggatcgcagtggtgagtaaccatgcatcatcaggagtacggataaaatgcttgatggtcggaagaggcataaattccgtcagccagtttagtctgaccatctcatctgtaacatcattggcaacgctacctttgccatgtttcagaaacaactctggcgcatcgggcttcccatacaatcggtagattgtcgcacctgattgcccgacattatcgcgagcccatttatacccatataaatcagcatccatgttggaatttaatcgcggccttgagcaagacgtttcccgttgaatatggctcataacagaacttattatttccttcctcttttctacagtatttaaagataccccaagaagctaattataacaagacgaactccaattcactgttccttgcattctaaaaccttaaataccagaaaacagctttttcaaagttgttttcaaagttggcgtataacatagtatcgacggagccgattttgaaaccgcggtgatcacaggcagcaacgctctgtcatcgttacaatcaacatgctaccctccgcgagatcatccgtgtttcaaacccggcagcttagttgccgttcttccgaatagcatcggtaacatgagcaaagtctgccgccttacaacggctctcccgctgacgccgtcccggactgatgggctgcctgtatcgagtggtgattttgtgccgagctgccggtcggggagctgttggctggctggtggcaggatatattgtggtgtaaacataacgaattcgtctca

SEQ ID NO: 24 - DNA, 20976 bp, synthetic construct
  source 1..20976: mol_type = other DNA; plasmid = DNA construct O4 = pDGB3alpha1[pE8:UGT2:T35S-p35S:UGT709G1:T35S-p2A11:CCD2L:T35S-pNos:Hyg:T35S]
ggagtccctaatgatattgttcacgtaattaagttttgtggaagtgagagagtccaattttgataagaaaagagtcagaaaacgtaatattttaaaagtctaaatctttctacaaataagagcaaatttatttattttttaatccaataaatattaatggaggacaaattcaattcacttggttgtaaaataaacttaaaccaataaccaaagaactaataaatcctgaagtggaattattaaggataaatgtacatagacaatgaagaaataataggttcgatgaattaataataattaaggatgttacaatcatcatgtgccaagtatatacacaatattctatgggatttataatttcgttacttcacttaacttttgcgtaaataaaacgaattatctgatattttataataaaacagttataagaaccatcatttttaacaacatagatatattatttctaatagtttaatgatacttttaaatcttttaaattttatgtttcttttagaaaataaaaattcaaaaaattaaatatatttacaaaaactacaatcaaacacaacttcatatattaaaagcaaaatatattttgaaaatttcaagtgtcctaacaaataagacaagaggaaaatgtacgatgagagacataaagagaactaataattgaggagtcctataatatataataaagtttattagtaaacttaattattaaggactcctaaaatatatgataggagaaaatgaatggtgagagatattggaaaacttaataattaaggattttaaaatatatggtaaaagataggcaaagtatccattatccccttttaacttgaagtctactaggcgcatgtgaaagttgattttttgtcacgtcatatagctataacgtaaaaaaagaaagtaaaatttttaattttttttaatatatgacatattttaaacgaaatataggacaaaatgtaaatgaatagtaaaggaaacaaagattaatacttactttgtaagaatttaagataaatttaaaatttaatagatcaactttacgtctagaaagacccatatctagaaggaatttcacgaaatcggcccttattcgaaaataacttttaaataatgaattttaaattttaagaaataatatccaatgaataaatgacatgtagcattttacctaaatatttcaactattttaatccaatattaatttgttttattcccaacaatagaaagtcttgtgcagacatttaatctgacttttccagtactaaatattaattttctgaagattttcgggtttagtccacaagttttagtgagaagttttgctcaaattttaggtgagaaggtttgatatttatcttttgttaaattaatttatctaggtgactattatttatttaagtagaaattcatatcattacttttgccaacttgtagtcataataggagtaggtgtatatgatgaaggaataaacaagttcagtgaagtgattaaaataaaatataatttaggtgtacatcaaataaaaaccttaaagtttagaaaggcaccgaataattttgcatagaagatattagtaaatttataaaaataaaagaaatgtagttgtcaagttgtcttcttttttttggataaaaatagcagttggcttatgtcattcttttacaacctccatgccacttgtccaattgttgacacttaactaattagtttgattcatgtatgaatactaaataattttttaggactgactcaaatatttttatattatcatagtaatatttatctaatttttaggaccacttattactaaataataaattaactacaactatattattgttgtgaaacaacaacgttttggttgttatgatgaaacgtacactatatcagtatgaaaaattcaaaacgattagtataaattatattgaaaatttgatatttttctattcttaatcagacgtattgggtttcatattttaaaaagggactaaacttagaagagaagtttgtttgaaactacttttgtctctttcttgttcccatttctctcttagatttcaaaaagtgaactactttatctccttctttgttcacattttattttattctattataaatatggcatcctcatattgagatttttagaaattattctaatcattcacagtgcaaaagaagaatgttgaacggcaacaaatgccacatcctcctcctcccctgtccagcacaaggccatatcaaccccattctccaattcggcaagcgactggcctctcacaacctcctcaccacactcgtcaacacccggttcctctccaactcgaccaaatccgaacccggtccggtcaacatccagtgcatatccgacggattcgatcccggtgggatgaatgcagcacctagtcgtcgggcctatttcgaccgacctcagagtcggtcgggtcagaaacatgttggcctcatcgagtcactccggtccagaggccgacccggcgcatgttttggtctacgacccgttcccctctgggcaatgaacgtagccgagcggtccgggctgcggtcggtcgcattctttactcagccgtgtgcagtggacacaatctaccgccacgtgtgggagggacgaattaaggttccggttgccgagccggtccggttgcctggattgcccccactcgagcctagtgatctgccgtgcgttcgtaacggattcggacgagtcgttaacccggatctcttgccacttcgagtgaatcagcacaaaaatttggacaaagctgacatgatggggaggaactccatatacgagctagaggcggatttgttggatgggtcccgattaccattaccggtgaagtcgattgggccgaccgtgccgtctacttatctcgacaaccgaatcccgtcggattcacactatggattcaatctatacacccctgacactactccctacttggactggctcgactccaaggccccgaactctgtcatctatgtctcatttggtagtttgtccagtctgagccctgatcaaaccaatgagattgcgtcgggtctgatcgccaccaacaaaagctttatttgggtggtacgcacttcggagttagccaaactccctgccaacttcacccaagagaatgcgagccgtgggctggttgtgacctggtgcgaccaactcgatctcctcgcacacgttgcgaccggttgcttcgtgactcactgcggatggaactcgactatggaaggtgtcgcacttggtgtgccgatggtgggagtgccgcagtggtcggaccagcctatgaatgccaagtatgtagaggatgtgtggaaggtcggcgtgagggcgaagacttatgggaaggattttgtgagaggggaggagttcaaaagatgtgtggaggaggtgatggatggagagaggagtggaaagattagagagaatgccgcaaggtggtgtaagttggccaaggactctgttagtgagggtgggagttctgacaagtgtatcaaggagttcatacatcagtgttgcaatgactccaaaatttccttagtttaagcttcggccatgctagagtccgcaaaaatcaccagtctctctctacaaatctatctctctctatttttctccagaataatgtgtgagtagttcccagataagggaattagggttcttatagggtttcgctcatgtgttgagcatataagaaacccttagtatgtatttgtatttgtaaaatacttctatcaataaaatttctaattcctaaaaccaaaatccagtgacctcgctgtcaggagactagagccaagctgatctcctttgccccggagatcaccatggacgactttctctatctctacgatctaggaagaaagttcgacggagaaggtgacgataccatgttcaccaccgataatgagaagattagcctcttcaatttcagaaagaatgctgacccacagatggttagagaggcctacgcggcaggtctgatcaagacgatctacccgagtaataatctccaggagatcaaataccttcccaagaaggttaaagatgcagtcaaaagattcaggactaactgcatcaagaacacagagaaagatatatttctcaagatcagaagtactattccagtatggacgattcaaggcttgcttcataaaccaaggcaagtaatagagattggagtctctaagaaagtagttcctactgaatcaaaggccatggagtcaaaaattcagatcgaggatctaacagaactcgccgtgaagactggcgaacagttcatacagagtcttttacgactcaatgacaagaagaaaatcttcgtcaacatggtggagcacgacactctcgtctactccaagaatatcaaagatacagtctcagaagaccaaagggctattgagacttttcaacaaagggtaatatcgggaaacctcctcggattccattgcccagctatctgtcacttcatcaaaaggacagtagaaaaggaaggtggcacctacaaatgccatcattgcgataaaggaaaggctatcgttcaagatgcctctgccgacagtggtcccaaagatggacccccacccacgaggagcatcgtggaaaaagaagacgttccaaccacgtcttcaaagcaagtggattgatgtgatatctccactgacgtaagggatgacgcacaatcccactatccttcgcaagacccttcctctatataaggaagttcatttcatttggagaggactccggtatttttacaacaataccacaacaaaacaaacaacaaacaacattacaatttactattctagtcgaaatggctgagaaagaagcaaatacccatgtcgtcctcttccccttgccaggccaagggcacatcggctcaatgttgaaactggcacagcttctttccaccgccggattctacgtcactttcgtccacaccgaacgcaactaccgtcgctacctcctcacctccacgtccttccacgtccccaagttccggttccgcaccatccccgacggttttcccgacgacgattcccgctcgcccctcccttttctcgagctccaagagtcgctggacacgaaatgtcgggggcattatcgggaattgttggtcgctgtcgacgaccaagaagagtggcccccagtcacttgtgtcgtggctgatcaagctcttccactctcactcgaagttcccgacgagttggggattcctgtaatgatactcgcaccacacagtgcgtgcagtatattgacgagttattcgattccggagcttataaggggaggtgaactccctatcccagatggggccaatatggatgaactattacaaggcgtactgggattggaaggtatcgtgaggcgtagggatatgtccatcagaagcgccaagtccatccaagatccatttcttcaattcgaagtgaaaatgagcaaaaacttgcccagaggaagagctctcatcctgaacactacagaatcgatagactctctttctttgcgacacattcggtcgatctgtcccactacctacgcactcgggcccttccacgtccttctcaggaacataaaagacgagtcccactccgcaagcctttccgaagaggacaggtcctgcatcgcctggctggactcgaaaccgaacaagtccgcggtctacgtgagtttcggtagcctcgccgccatggcgagagaagcatttcttgagtttcagcagggattgctcgacagcgggtattacttcttgtgggtgatccggcccgatatggtggaaggggggctggaagagagcgagctgaccgcgagcgaacaacgctactttgtgaagtgggccccacaggaggaggttcttgcgcacccggcggtagggtgtttcttgacgcacagcggttggaactctacgttggagagtatctttgcgggagtgccgatgatatgttggcctttctttgcggaccagctgattaacagtaggtttgcgagcgaggtgtggaaaattgccttggatatgaaggatttgtgcggaaggagccacgtggagaggatggtgaaggaagttatgagtggagagaaaggcgaagagctaaggaattctagctgcgagatggcagatagggtgaagaagagtgcagaggaaggtggctcttcctacgccaacttcaaagagttggttggacatatcaaatctttgagcttaccagcagaaagaggagaaaatggtggtgaaggaatgagtgtacaagcgccgagtaaacttttcctcctcaacgctgaggacggaaaacatgtccttaaaagtgacgaaccgtcggaacaaaggggtccacaatttaatccaaattttcttcggacctgagcttcggccatgctagagtccgcaaaaatcaccagtctctctctacaaatctatctctctctatttttctccagaataatgtgtgagtagttcccagataagggaattagggttcttatagggtttcgctcatgtgttgagcatataagaaacccttagtatgtatttgtatttgtaaaatacttctatcaataaaatttctaattcctaaaaccaaaatccagtgacctcgctgtcaggagagcgcgagtcggtcccattattgaagcatttatcagggttattgtctcatgagcggatacatatttgaatgtatttagaaaaataaacaaataggggttccgcgcacatttccccgaaaagtgccacctgacgtctaagaaaccattattatcatgacattaacctataaaaataggcgtatcacgaggccctttcgtcttcaagaattagcttggcaattcccgatctagtaacatagatgacaccghgcgcgataatttatcctagtttgcgcgctatattttgttttctatcgcgtattaaatgtataattgcgggactctaatcataaaaacccatctcataaataacgtcatgcattacatgttaattattacatgcttaacgtaattcaacagaaattatatgataatcgtcgcaagaccggcaacaggattcaatcttaagaaactttattgccaaatgtttgaacgatcgggatcgaagatccattccaagctcattcctttgccctcggacgagtgctggggcgtcggtttccactatcggcgagtacttctacacagccatcggtccagacggccgcgcttctgcgggcgatttgtgtacgcccgacagtcccggctccggatcggacgattgcgtcgcatcgaccctgcgcccaagctgcatcatcgaaattgccgtcaaccaagctctgatagagttggtcaagaccaatgcggagcatatacgcccggagtcgtggcgatcctgcaagctccggatgcctccgctcgaagtagcgcgtctgctgctccatacaagccaaccacggcctccagaagaagatgttggcgacctcgtattgggaatccccgaacattgcctcgctccagtcaatgaccgctgttatgcggccattgtccgtcaggacattgttggagccgaaatccgcgtgcacgaggtgccggacttcggggcagtcctcggcccaaagcatcagctcatcgagagcctgcgcgacggacgcactgacggtgtcgtccatcacagtttgccagtgatacacatggggatcagcaatcgcgcatatgaaatcacgccatgtagtgtattgaccgattccttgcggtccgaatgggccgaacccgctcgtctggctaagatcggccgcagcgatcgcatccatggcctccgcgaccggctgcagaacagcgggcagttcggtttcaggcaggtcttgcaacgtgacaccctgtgcacggcgggagatgcaataggtcaggctctcgctgaattccccaatgtcaagcacttccggaatcgggagcgcggccgatgcaaagtgccgataaacataacgatctttgtagaaaccatcggcgcagctatttacccgcaggacatatccacgccctcctacatcgaagctgaaagcacgagattcttcgccctccgagagctgcatcaggtcggacacgctgtcgaacttttcgatcagaaacttctcgacagacgtcgcggtgagttcaggctttttcattgcctcgatcgagttgagagtgaatatgagactctaattggataccgaggggaatttatggaacgtcagtggagcatttttgacaagaaatatttgctagctgatagtgaccttaggcgacttttgaacgcgcaataatggtttctgacgtatgtgcttagctcattaaactccagaaacccgcggctcagtggctccttcaacgttgcggttctgtcagttccaaacgtaaaacggcttgtcccgcgtcatcggcgggggtcataccgtgactcccttaattctcatgtatctccgtcaggaggtcaaacaattttgaggaattcaatttcatctttaactggtacaataatcattttatcatgaaaataagcagctcaagagaatttttgaagaatcttttatttctttaacatttaaccacatgaatttttaatttttttttgcaatacatttaaaccgaaatggtcaaacgatcaaccaactgatctttattctaataaacttctagtttacatttgcatgtgagtgcatcatcattatcatatttgtacacaacaaacaagaaaaaaatataaacaatattttatttaaatatttatattccactttgactgtagatattaaatcttgtcatcatttatagtctcaatattataatttttttattttttcaaaattcaaaagtttacaattatttttttgaactataatattatccaagatgaacatctcaagaagaaaattattaatattgttatggttaaaattttacatacaatacttgttttttgctttacttttatcttaccgtagatacacaatcgacgataacttagtgatcacacaataataattattttgttcatgacacaatatttataagaaatacttatttctttcttttatccttcagtagttcataataaaaacataccataatatttgtgatgcattcatagtacgtaatgaaatgacaatttatgtcaaattattttcttttatactctcaaacctcccgtaaaggtgagatgagtcatttatccaattatacataaatatgtctttattcatgctctttatcacattctgacacattcacttaatttcaagagtaagcaagcatgataactgaaactatttatgcgtatcttaccttgatatttgacacattacatgacacacctcaacatcactttcaaagattaagcgcaccaccatattatctttctttttttttttatgaaggttttataaaattattaaattaggtccaaaaaattgtttgtcaaataaccttttatactagattgatgacaaaaattacctttacgttttgaaagaccattttaagacctaatctatcagtgactccttaaagttggcacaatatttcacttagacaccctaattgaatgatgttcattttaaacacccaatgtagggttccgctatatcattttgacacatttcttaacatcaacaaaaatatataatgagtatgtgatatactcgcgaatgacgtgaaaaatgaagacatttgttatttgtatcaaagtagttactaaataattaattttgaataaaaataaaagctgaccagtaaatcaataacacataatattttccacctaataattaaaatataaaataaaaaagagccatctcagggtcatctgcccaccattgctatttcaaagaaatttgtacgttagtttatagaaattgatgttaaaattctttcaagaaaaatttatgaatgaatttattctctaatttaaaaatattttctgttatttttgttgaaagaaatttaacttggataaaatggtggttaaaactggaaagaagaaaagagaaaaaataattaaaaatcatttcacgctctaatcaatgagcgtatcacattcattatgttatataagcaaaagtgacaaaacgaaaataatatattacatgaaatgtctaaaataaatatcgtctaattaaaatatctaagtaacatattgtgcctaactttagagggatcatcaataagttaaaccccattttaataactcataattgtcctttttatttaatattgtcacaaatcacaatgataattaacattaatttgtcctttgtgacgtccatattcatgcatttaaccaatcatcttcatttggacttattatcacaattatcccactttcctcacaaaatggagcattcaagtggaatagactacacgatttttaatttcatcaaaaacatctttttgctttattcattattatattgtcgctattgttgaattttatttgccctaaatttcttaccataaatagatttttcttttagaaaaaggagattgactaattcttttcttgtaggaaaaggtttaggactctataaatagagacatattccttctaacttaatcaacatttacaatgtagtcttaaagactttgaaagtttttggttagggggagaaattgtgggtcacaagcttgatacgttatcaattgtgtaaacctcccatgtattctgagtgaatttggttgaggttgtttccctctgtattttgtactctcatatttatagtggattgttcatctctttcgtggacgtaggtcgattgaccgtcgattgaccgaaccacgttaaatctttgtattttttgatatatttctcattatcttcttactcgtgatctttcaaggtttgcattgctatcttccgcgttacaccaacttatttacgatcctaacagctatggtgtggaaacataaatcaaacattttactgatataaacacatctttgattataacatgatagaaatttgagcccaactttttatcatcattatatacaaaaagttctaaattttttttttgatgtagtaaaacttaaatccatagtcttgcccctaaaccaatgacataatatataacccaaaatatactagttttcgccctcgagccctttaaaaagtatagtcaatatttacggtgaccgtgaatttcttaattatgatatataatttaaaagaaatcatgatcacattctactgatgagaacatgtgctaatcaagggaaaacatggatgtgaaaaatactttttgttaaaagtaaaaaaaaatgtgaaattttgttagttatttactacctatacattatttgagcatgtgcaaactttacaaatacctaatagaagattttcacctgcctgtatatatgtaaattaattataatgaacactctcacataaaataattatcagtatatacattaatacttgccctccacaatgaattaaataaaatgtagaacatgatctacacttcaataaaactaagaccataaagaataatttcaaaatatacacatgtcaacaataaattatttgcatattatattaacttactaaacaatctttacttttgaaatataaaaataatcaagttataagtctgctcaaagtaaagcacttgttagactcatctgattttgagaaggtaagcaaattgatggtgcataatagtcacaagtaaaatataaaatagatttcattagtaaaattgttttttactttctttatatataattatcaatatccttcaatggtaggttaattatattgttaacttcttgttgaattaaagcaataagacaagaatattaaagataaaagaacaataaaaatagaaagactaagagataagagttttcttattcttctttcaataagtatcatcaagtgtatacaatataaatttttgtatttttgatctatctatttataatgttatatataagcatacaaaagatcagtcataaatatgactttaatcatgaaaataatgaaagagattatgaaggcgtaaggttactagaataatagtcattaaaaaaaggggttatctttataattgaataattgatgaagtaatggagataattagtgagcataaatttttttaaaaaaatggacatttacactataatattttataacactttcccttaaacatctaggtataaataatgagtcttgtcaaaatcttagtaggaaaaattctgtgaaatttttttagtgaaaacaaatgatataaatatcttgaatactcattatttgttgtctcattaaaaatcttatctgacctataaaataaattatttgctcaactcaaaatagtttttcattctaaaattagtataattattagtgaatatttaattaacataattgtatactaaggggcctataaattggattcttctcaaagaaaaataaaatcaccacacaactttcttcttctgctcatcaattagcaattaatccaaaaccaaatggaatctcctgctactaaattacctgcacctctgctgatgttatcttcttctccattccttctcccttctcctaataagagctcctccatcttccttccacgtaaattagggccgctacctccaaaatattattattacaattgctgccatcctaagagtagatcaatctcagtagtatcaatggcaaataaggaggaggcagagacaagtaagaagaagcccaaaccattaaaagtactaattaccaaagtggatccgaagccgaggaagggcatggcatccgtcgcagtggacttactcgagaaggcctttgtatacctattgtccggaaattctgcagctgatcgtagtagtagtagtggtcgtcgtcgtcgtaaagagcattactacctctccggcaattatgcgcccgtcggacacgaaaccccgccctccgaccacctccccattcatggatcccttcctgaatgcttgaatggagtgtttctgagagttggtcctaaccccaagtttgctcccgtagccggatacaattgggtcgatggagatggaatgattcatggattgcgtattaaagatggaaaagcaacttatctatctcgatatattaaaacgtcacggtttaaacaagaagaatattttggaagagcaaaatttatgaagattggagatctaaggggattgcttgggttctttacgatcttaatactagtacttcgaacaacattgaaagtaatagacatttcatatggaagagggacgggtaatacagctcttgtgtatcataatggcttactattggctctatcagaagaagataaaccttatgttgttaaagttttagaagatggagacttgcaaactcttgggatattggattatgacaagaaattgtcacatccattcaccgctcatccaaagatcgatccgttaactgatgagatgtttacctttggatattccatctcgcctccgtatcttacttatcgagtcatttccaaggatggagtgatgcaagatccagtgcaaatctcaattacatcccctaccataatgcatgattttgctattactgaaaattatgccatcttcatggacctgcccttgtatttccaaccagaggaaatggtaaaggggaaatttgtctcttcatttcaccctacaaaaagagctcgtatcggtgtgcttccacgatatgcaaaagacgagcatccaattcgatggttcgatcttccaagttgcttcatgactcataatgcaaatgcttgggaagagaatgatgaagttgtgctattcacatgtcgccttgagagtcctgatcttgacatgcttagtggacctgcggaagaagagattgggaattcaaaaagtgagctttacgaaatgaggttcaatttgaaaactggaattacttcacaaaagcaactatctgtacctagtgttgattttcctcggatcaaccaaagttatactggcaggaaacagcaatatgtttattgtactcttggcaacaccaagattaagggcattgtgaagtttgatctgcaaattgaaccagaagccggaaagacaatgcttgaagttggaggaaatgtacaaggcatctttgagttgggacctagaagatatggttcagaggcaatatttgtgccatgccaacctggcatcaaatctgatgaggatgacggttacttgatattctttgtacacgacgaaaacaatgggaaatctgaggtcaatgtcatcgatgcaaagacaatgtctgcagaacctgtggctgttgtggaacttccaagcagggttccatatggattccatgccttgtttctgaatgaggaagaacttcagaagcaccaagcagagacatgagcttcggccatgctagagtccgcaaaaatcaccagtctctctctacaaatctatctctctctatttttctccagaataatgtgtgagtagttcccagataagggaattagggttcttatagggtttcgctcatgtgttgagcatataagaaacccttagtatgtatttgtatttgtaaaatacttctatcaataaaatttctaattcctaaaaccaaaatccagtgacctcgctgtcatgagacgaattctgacaggatatattggcgggtaaacctaagagaaaagagcgtttattagaataatcggatatttaaaagggcgtgaaaaggtttatccgttcgtccatttgtatgtgcatgccaaccacagggttcccctcgggatcaaagtactttgatccaacccctccgctgctatagtgcagtcggcttctgacgttcagtgcagccgtcatctgaaaacgacatgtcgcacaagtcctaagttacgcgacaggctgccgccctgcccttttcctggcgttttcttgtcgcgtgttttagtcgcataaagtagaatacttgcgactagaaccggagacattacgccatgaacaagagcgccgccgctggcctgctgggctatgcccgcgtcagcaccgacgaccaggacttgaccaaccaacgggccgaactgcacgcggccggctgcaccaagctgttttccgagaagatcaccggcaccaggcgcgaccgcccggagctggccaggatgcttgaccacctacgccctggcgacgttgtgacagtgaccaggctagaccgcctggcccgcagcacccgcgacctactggacattgccgagcgcatccaggaggccggcgcgggcctgcgtagcctggcagagccgtgggccgacaccaccacgccggccggccgcatggtgttgaccgtgttcgccggcattgccgagttcgagcgttccctaatcatcgaccgcacccggagcgggcgcgaggccgccaaggcccgaggcgtgaagtttggcccccgccctaccctcaccccggcacagatcgcgcacgcccgcgagctgatcgaccaggaaggccgcaccgtgaaagaggcggctgcactgcttggcgtgcatcgctcgaccctgtaccgcgcacttgagcgcagcgaggaagtgacgcccaccgaggccaggcggcgcggtgccttccgtgaggacgcattgaccgaggccgacgccctggcggccgccgagaatgaacgccaagaggaacaagcatgaaaccgcaccaggacggccaggacgaaccgtttttcattaccgaagagatcgaggcggagatgatcgcggccgggtacgtgttcgagccgcccgcgcacctctcaaccgtgcggctgcatgaaatcctggccggtttgtctgatgccaagctggcggcctggccggccagcttggccgctgaagaaaccgagcgccgccgtctaaaaaggtgatgtgtatttgagtaaaacagcttgcgtcatgcggtcgctgcgtatatgatccgatgagtaaataaacaaatacgcaaggggaacgcatgaaggttatcgctgtacttaaccagaaaggcgggtcaggcaagacgaccatcggaacccatctagcccgcgccctgcaactcgccggggccgatgttctgttagtcgattccgatccccagggcagtgcccgcgattgggcggccgtgcgggaagatcaaccgctaaccgttgtcggcatcgaccgcccgacgattgaccgcgacgtgaaggccatcggccggcgcgacttcgtagtgatcgacggagcgccccaggcggcggacttggctgtgtccgcgatcaaggcagccgacttcgtgctgattccggtgcagccaagcccttacgacatatgggccaccgccgacctggtggagctggttaagcagcgcattgaggtcacggatggaaggctacaagcggcctttgtcgtgtcgcgggcgatcaaaggcacgcgcatcggcggtgaggttgccgaggcgctggccgggtacgagctgcccattcttgagtcccgtatcacgcagcgcgtgagctacccaggcactgccgccgccggcacaaccgttcttgaatcagaacccgagggcgacgctgcccgcgaggtccaggcgctggccgctgaaattaaatcaaaactcatttgagttaatgaggtaaagagaaaatgagcaaaagcacaaacacgctaagtgccggccgtccgagcgcacgcagcagcaaggctgcaacgttggccagcctggcagacacgccagccatgaagcgggtcaactttcagttgccggcggaggatcacaccaagctgaagatgtacgcggtacgccaaggcaagaccattaccgagctgctatctgaatagatcgcgcagctaccagagtaaatgagcaaatgaataaatgagtagatgaattttagcggctaaaggaggcggcatggaaaatcaagaacaaccaggcaccgacgccgtggaatgccccatgtgtggaggaacgggcggttggccaggcgtaagcggctgggttgtctgccggccctgcaatggcactggaacccccaagcccgaggaatcggcgtgacggtcgcaaaccatccggcccggtacaaatcggcgcggcgctgggtgatgacctggtggagaagttgaaggccgcgcaggccgcccagcggcaacgcatcgaggcagaagcacgccccggtgaatcgtggcaagcggccgctgatcgaatccgcaaagaatcccggcaaccgccggcagccggtgcgccgtcgattaggaagccgcccaagggcgacgagcaaccagattttttcgttccgatgctctatgacgtgggcacccgcgatagtcgcagcatcatggacgtggccgttttccgtctgtcgaagcgtgaccgacgagctggcgaggtgatccgctacgagcttccagacgggcacgtagaggtttccgcagggccggccggcatggccagtgtgtgggattacgacctggtactgatggcggtttcccatctaaccgaatccatgaaccgataccgggaagggaagggagacaagcccggccgcgtgttccgtccacacgttgcggacgtactcaagttctgccggcgagccgatggcggaaagcagaaagacgacctggtagaaacctgcattcggttaaacaccacgcacgttgccatgcagcgtacgaagaaggccaagaacggccgcctggtgacggtatccgagggtgaagccttgattagccgctacaagatcgtaaagagcgaaaccgggcggccggagtacatcgagatcgagctagctgattggatgtaccgcgagatcacagaaggcaagaacccggacgtgctgacggttcaccccgattactttttgatcgatcccggcatcggccgttttctctaccgcctggcacgccgcgccgcaggcaaggcagaagccagatggttgttcaagacgatctacgaacgcagtggcagcgccggagagttcaagaagttctgtttcaccgtgcgcaagctgatcgggtcaaatgacctgccggagtacgatttgaaggaggaggcggggcaggctggcccgatcctagtcatgcgctaccgcaacctgatcgagggcgaagcatccgccggttcctaatgtacggagcagatgctagggcaaattgccctagcaggggaaaaaggtcgaaaaggactctttcctgtggatagcacgtacattgggaacccaaagccgtacattgggaaccggaacccgtacattgggaacccaaagccgtacattgggaaccggtcacacatgtaagtgactgatataaaagagaaaaaaggcgatttttccgcctaaaactctttaaaacttattaaaactcttaaaacccgcctggcctgtgcataactgtctggccagcgcacagccgaagagctgcaaaaagcgcctacccttcggtcgctgcgctccctacgccccgccgcttcgcgtcggcctatcgcggccgctggccgctcaaaaatggctggcctacggccaggcaatctaccagggcgcggacaagccgcgccgtcgccactcgaccgccggcgcccacatcaaggcaccctgcctcgcgcgtttcggtgatgacggtgaaaacctctgacacatgcagctcccggtgacggtcacagcttgtctgtaagcggatgccgggagcagacaagcccgtcagggcgcgtcagcgggtgttggcgggtgtcggggcgcagccatgacccagtcacgtagcgatagcggagtgtatactggcttaactatgcggcatcagagcagattgtactgagagtgcaccatatgcggtgtgaaataccgcacagatgcgtaaggagaaaataccgcatcaggcgctcttccgcttcctcgctcactgactcgctgcgctcggtcgttcggctgcggcgagcggtatcagctcactcaaaggcggtaatacggttatccacagaatcaggggataacgcaggaaagaacatgtgagcaaaaggccagcaaaaggccaggaaccgtaaaaaggccgcgttgctggcgtttttccataggctccgcccccctgacgagcatcacaaaaatcgacgctcaagtcagaggtggcgaaacccgacaggactataaagataccaggcgtttccccctggaagctccctcgtgcgctctcctgttccgaccctgccgcttaccggatacctgtccgcctttctcccttcgggaagcgtggcgctttctcatagctcacgctgtaggtatctcagttcggtgtaggtcgttcgctccaagctgggctgtgtgcacgaaccccccgttcagcccgaccgctgcgccttatccggtaactatcgtcttgagtccaacccggtaagacacgacttatcgccactggcagcagccactggtaacaggattagcagagcgaggtatgtaggcggtgctacagagttcttgaagtggtggcctaactacggctacactagaaggacagtatttggtatctgcgctctgctgaagccagttaccttcggaaaaagagttggtagctcttgatccggcaaacaaaccaccgctggtagcggtggtttttttgtttgcaagcagcagattacgcgcagaaaaaaaggatctcaagaagatcctttgatcttttctacggggtctgacgctcagtggaacgaaaactcacgttaagggattttggtcatgcattctaggtgattagaaaaactcatcgagcatcaaatgaaactgcaatttattcatatcaggattatcaataccatatttttgaaaaagccgtttctgtaatgaaggagaaaactcaccgaggcagttccataggatggcaagatcctggtatcggtctgcgattccgactcgtccaacatcaatacaacctattaatttcccctcgtcaaaaataaggttatcaagtgagaaatcaccatgagtgacgactgaatccggtgagaatggcaaaagtttatgcatttctttccagacttgttcaacaggccagccattacgctcgtcatcaaaatcactcgcatcaaccaaaccgttattcattcgtgattgcgcctgagcgagtcgaaatacgcgatcgctgttaaaaggacaattacaaacaggaatcgaatgcaaccggcgcaggaacactgccagcgcatcaacaatattttcacctgaatcaggatattcttctaatacctggaatgctgttttccctgggatcgcagtggtgagtaaccatgcatcatcaggagtacggataaaatgcttgatggtcggaagaggcataaattccgtcagccagtttagtctgaccatctcatctgtaacatcattggcaacgctacctttgccatgtttcagaaacaactctggcgcatcgggcttcccatacaatcggtagattgtcgcacctgattgcccgacattatcgcgagcccatttatacccatataaatcagcatccatgttggaatttaatcgcggccttgagcaagacgtttcccgttgaatatggctcataacagaacttattatttccttcctcttttctacagtatttaaagataccccaagaagctaattataacaagacgaactccaattcactgttccttgcattctaaaaccttaaataccagaaaacagctttttcaaagttgttttcaaagttggcgtataacatagtatcgacggagccgattttgaaaccgcggtgatcacaggcagcaacgctctgtcatcgttacaatcaacatgctaccctccgcgagatcatccgtgtttcaaacccggcagcttagttgccgttcttccgaatagcatcggtaacatgagcaaagtctgccgccttacaacggctctcccgctgacgccgtcccggactgatgggctgcctgtatcgagtggtgattttgtgccgagctgccggtcggggagctgttggctggctggtggcaggatatattgtggtgtaaacataacgaattcgtctca

SEQ ID NO: 25 - DNA, 21 bp, synthetic construct
  source 1..21: mol_type = other DNA; note = CsUGT2 forward primer
tcgagcctagtgatctgccgt

SEQ ID NO: 26 - DNA, 21 bp, synthetic construct
  source 1..21: mol_type = other DNA; note = CsUGT2 reverse primer
tcgagccagtccaagtaggga

SEQ ID NO: 27 - DNA, 22 bp, synthetic construct
  source 1..22: mol_type = other DNA; note = UGT709G1 forward primer
actcacctccacgtccttccag

SEQ ID NO: 28 - DNA, 21 bp, synthetic construct
  source 1..21: mol_type = other DNA; note = UGT709G1 reverse primer
cttgatcagccacgacacaag

SEQ ID NO: 29 - DNA, 20 bp, synthetic construct
  source 1..20: mol_type = other DNA; note = CsCCD2L forward primer
acatgtcgccttgagagtcc

SEQ ID NO: 30 - DNA, 20 bp, synthetic construct
  source 1..20: mol_type = other DNA; note = CsCCD2L reverse primer
tcagatttgatgccaggttg

SEQ ID NO: 31 - DNA, 21 bp, synthetic construct
  source 1..21: mol_type = other DNA; note = Actin-2 forward primer
cattgtgctcagtggtggttc

SEQ ID NO: 32 - DNA, 21 bp, synthetic construct
  source 1..21: mol_type = other DNA; note = Actin-2 reverse primer
tctgctggaaggtgctaagtg

SEQ ID NO: 33 - DNA, 635 bp, synthetic construct
  source 1..635: mol_type = other DNA; note = pPat promoter
aatttgtcaaatcaggctcaaagatcgtttttcatatcggaatgaggattttatttattcttttaaaaataaagaggtggtgactaaacaatttcaaatctcatcacacatatggggtcagcccacaaaaataaagaacggtggaacggactgatatataatactaataaagaataggaaaaggaaagtgagtgaggtgcgagggagagaatttgtttaatatcagagtcgatcatgtgtcagttttatcgatatgattctgacttcaactgagtttaagcaattctgataaggcggagaaaatcatagtgctgagtctagaaaaatctcatgcagtgtgagataaacctcaaacaagaacatttgcggtgctaaacaatttcaagtcttatcacacatatatattatatattactaataaagaatagaaaaaggaaaggtaaacatcactaatgacagttgcggtgcaaagtgagtgagataataaacatcactaatagacatcactaacttttattggttatgtcaaactcaaaataaaatttctcaacttgtttacgtgcctatatataccatgcttgttatatgctcaaagcaccaaacaaaatttaaaaacactttgaacatttgcaaag

SEQ ID NO: 34 - DNA, 15632 bp, synthetic construct
  source 1..15632: mol_type = other DNA; plasmid = DNA construct O6 = pDGB3alpha2[pPatGT2T35S-pPatUGT709T35S-pPatCCD2LT35S-pNos-Hyg-T35S]
ggagagcgcgagtcggtcccattattgaagcatttatcagggttattgtctcatgagcggatacatatttgaatgtatttagaaaaataaacaaataggggttccgcgcacatttccccgaaaagtgccacctgacgtctaagaaaccattattatcatgacattaacctataaaaataggcgtatcacgaggccctttcgtcttcaagaattagcttggcaattcccgatctagtaacatagatgacaccghgcgcgataatttatcctagtttgcgcgctatattttgttttctatcgcgtattaaatgtataattgcgggactctaatcataaaaacccatctcataaataacgtcatgcattacatgttaattattacatgcttaacgtaattcaacagaaattatatgataatcgtcgcaagaccggcaacaggattcaatcttaagaaactttattgccaaatgtttgaacgatcgggatcgaagatccattccaagctcattcctttgccctcggacgagtgctggggcgtcggtttccactatcggcgagtacttctacacagccatcggtccagacggccgcgcttctgcgggcgatttgtgtacgcccgacagtcccggctccggatcggacgattgcgtcgcatcgaccctgcgcccaagctgcatcatcgaaattgccgtcaaccaagctctgatagagttggtcaagaccaatgcggagcatatacgcccggagtcgtggcgatcctgcaagctccggatgcctccgctcgaagtagcgcgtctgctgctccatacaagccaaccacggcctccagaagaagatgttggcgacctcgtattgggaatccccgaacattgcctcgctccagtcaatgaccgctgttatgcggccattgtccgtcaggacattgttggagccgaaatccgcgtgcacgaggtgccggacttcggggcagtcctcggcccaaagcatcagctcatcgagagcctgcgcgacggacgcactgacggtgtcgtccatcacagtttgccagtgatacacatggggatcagcaatcgcgcatatgaaatcacgccatgtagtgtattgaccgattccttgcggtccgaatgggccgaacccgctcgtctggctaagatcggccgcagcgatcgcatccatggcctccgcgaccggctgcagaacagcgggcagttcggtttcaggcaggtcttgcaacgtgacaccctgtgcacggcgggagatgcaataggtcaggctctcgctgaattccccaatgtcaagcacttccggaatcgggagcgcggccgatgcaaagtgccgataaacataacgatctttgtagaaaccatcggcgcagctatttacccgcaggacatatccacgccctcctacatcgaagctgaaagcacgagattcttcgccctccgagagctgcatcaggtcggacacgctgtcgaacttttcgatcagaaacttctcgacagacgtcgcggtgagttcaggctttttcattgcctcgatcgagttgagagtgaatatgagactctaattggataccgaggggaatttatggaacgtcagtggagcatttttgacaagaaatatttgctagctgatagtgaccttaggcgacttttgaacgcgcaataatggtttctgacgtatgtgcttagctcattaaactccagaaacccgcggctcagtggctccttcaacgttgcggttctgtcagttccaaacgtaaaacggcttgtcccgcgtcatcggcgggggtcataccgtgactcccttaattctcatgtatctccgtcaggagaatttgtcaaatcaggctcaaagatcgtttttcatatcggaatgaggattttatttattcttttaaaaataaagaggtggtgactaaacaatttcaaatctcatcacacatatggggtcagcccacaaaaataaagaacggtggaacggactgatatataatactaataaagaataggaaaaggaaagtgagtgaggtgcgagggagagaatttgtttaatatcagagtcgatcatgtgtcagttttatcgatatgattctgacttcaactgagtttaagcaattctgataaggcggagaaaatcatagtgctgagtctagaaaaatctcatgcagtgtgagataaacctcaaacaagaacatttgcggtgctaaacaatttcaagtcttatcacacatatatattatatattactaataaagaatagaaaaaggaaaggtaaacatcactaatgacagttgcggtgcaaagtgagtgagataataaacatcactaatagacatcactaacttttattggttatgtcaaactcaaaataaaatttctcaacttgtttacgtgcctatatataccatgcttgttatatgctcaaagcaccaaacaaaatttaaaaacactttgaacatttgcaaagaatggaatctcctgctactaaattacctgcacctctgctgatgttatcttcttctccattccttctcccttctcctaataagagctcctccatcttccttccacgtaaattagggccgctacctccaaaatattattattacaattgctgccatcctaagagtagatcaatctcagtagtatcaatggcaaataaggaggaggcagagacaagtaagaagaagcccaaaccattaaaagtactaattaccaaagtggatccgaagccgaggaagggcatggcatccgtcgcagtggacttactcgagaaggcctttgtatacctattgtccggaaattctgcagctgatcgtagtagtagtagtggtcgtcgtcgtcgtaaagagcattactacctctccggcaattatgcgcccgtcggacacgaaaccccgccctccgaccacctccccattcatggatcccttcctgaatgcttgaatggagtgtttctgagagttggtcctaaccccaagtttgctcccgtagccggatacaattgggtcgatggagatggaatgattcatggattgcgtattaaagatggaaaagcaacttatctatctcgatatattaaaacgtcacggtttaaacaagaagaatattttggaagagcaaaatttatgaagattggagatctaaggggattgcttgggttctttacgatcttaatactagtacttcgaacaacattgaaagtaatagacatttcatatggaagagggacgggtaatacagctcttgtgtatcataatggcttactattggctctatcagaagaagataaaccttatgttgttaaagttttagaagatggagacttgcaaactcttgggatattggattatgacaagaaattgtcacatccattcaccgctcatccaaagatcgatccgttaactgatgagatgtttacctttggatattccatctcgcctccgtatcttacttatcgagtcatttccaaggatggagtgatgcaagatccagtgcaaatctcaattacatcccctaccataatgcatgattttgctattactgaaaattatgccatcttcatggacctgcccttgtatttccaaccagaggaaatggtaaaggggaaatttgtctcttcatttcaccctacaaaaagagctcgtatcggtgtgcttccacgatatgcaaaagacgagcatccaattcgatggttcgatcttccaagttgcttcatgactcataatgcaaatgcttgggaagagaatgatgaagttgtgctattcacatgtcgccttgagagtcctgatcttgacatgcttagtggacctgcggaagaagagattgggaattcaaaaagtgagctttacgaaatgaggttcaatttgaaaactggaattacttcacaaaagcaactatctgtacctagtgttgattttcctcggatcaaccaaagttatactggcaggaaacagcaatatgtttattgtactcttggcaacaccaagattaagggcattgtgaagtttgatctgcaaattgaaccagaagccggaaagacaatgcttgaagttggaggaaatgtacaaggcatctttgagttgggacctagaagatatggttcagaggcaatatttgtgccatgccaacctggcatcaaatctgatgaggatgacggttacttgatattctttgtacacgacgaaaacaatgggaaatctgaggtcaatgtcatcgatgcaaagacaatgtctgcagaacctgtggctgttgtggaacttccaagcagggttccatatggattccatgccttgtttctgaatgaggaagaacttcagaagcaccaagcagagacatgagcttcggccatgctagagtccgcaaaaatcaccagtctctctctacaaatctatctctctctatttttctccagaataatgtgtgagtagttcccagataagggaattagggttcttatagggtttcgctcatgtgttgagcatataagaaacccttagtatgtatttgtatttgtaaaatacttctatcaataaaatttctaattcctaaaaccaaaatccagtgacctcgctgtcaggagaatttgtcaaatcaggctcaaagatcgtttttcatatcggaatgaggattttatttattcttttaaaaataaagaggtggtgactaaacaatttcaaatctcatcacacatatggggtcagcccacaaaaataaagaacggtggaacggactgatatataatactaataaagaataggaaaaggaaagtgagtgaggtgcgagggagagaatttgtttaatatcagagtcgatcatgtgtcagttttatcgatatgattctgacttcaactgagtttaagcaattctgataaggcggagaaaatcatagtgctgagtctagaaaaatctcatgcagtgtgagataaacctcaaacaagaacatttgcggtgctaaacaatttcaagtcttatcacacatatatattatatattactaataaagaatagaaaaaggaaaggtaaacatcactaatgacagttgcggtgcaaagtgagtgagataataaacatcactaatagacatcactaacttttattggttatgtcaaactcaaaataaaatttctcaacttgtttacgtgcctatatataccatgcttgttatatgctcaaagcaccaaacaaaatttaaaaacactttgaacatttgcaaagaatgttgaacggcaacaaatgccacatcctcctcctcccctgtccagcacaaggccatatcaaccccattctccaattcggcaagcgactggcctctcacaacctcctcaccacactcgtcaacacccggttcctctccaactcgaccaaatccgaacccggtccggtcaacatccagtgcatatccgacggattcgatcccggtgggatgaatgcagcacctagtcgtcgggcctatttcgaccgacctcagagtcggtcgggtcagaaacatgttggcctcatcgagtcactccggtccagaggccgacccggcgcatgttttggtctacgacccgttcccctctgggcaatgaacgtagccgagcggtccgggctgcggtcggtcgcattctttactcagccgtgtgcagtggacacaatctaccgccacgtgtgggagggacgaattaaggttccggttgccgagccggtccggttgcctggattgcccccactcgagcctagtgatctgccgtgcgttcgtaacggattcggacgagtcgttaacccggatctcttgccacttcgagtgaatcagcacaaaaatttggacaaagctgacatgatggggaggaactccatatacgagctagaggcggatttgttggatgggtcccgattaccattaccggtgaagtcgattgggccgaccgtgccgtctacttatctcgacaaccgaatcccgtcggattcacactatggattcaatctatacacccctgacactactccctacttggactggctcgactccaaggccccgaactctgtcatctatgtctcatttggtagtttgtccagtctgagccctgatcaaaccaatgagattgcgtcgggtctgatcgccaccaacaaaagctttatttgggtggtacgcacttcggagttagccaaactccctgccaacttcacccaagagaatgcgagccgtgggctggttgtgacctggtgcgaccaactcgatctcctcgcacacgttgcgaccggttgcttcgtgactcactgcggatggaactcgactatggaaggtgtcgcacttggtgtgccgatggtgggagtgccgcagtggtcggaccagcctatgaatgccaagtatgtagaggatgtgtggaaggtcggcgtgagggcgaagacttatgggaaggattttgtgagaggggaggagttcaaaagatgtgtggaggaggtgatggatggagagaggagtggaaagattagagagaatgccgcaaggtggtgtaagttggccaaggactctgttagtgagggtgggagttctgacaagtgtatcaaggagttcatacatcagtgttgcaatgactccaaaatttccttagtttaagcttcggccatgctagagtccgcaaaaatcaccagtctctctctacaaatctatctctctctatttttctccagaataatgtgtgagtagttcccagataagggaattagggttcttatagggtttcgctcatgtgttgagcatataagaaacccttagtatgtatttgtatttgtaaaatacttctatcaataaaatttctaattcctaaaaccaaaatccagtgacctcgctgtcaggagaatttgtcaaatcaggctcaaagatcgtttttcatatcggaatgaggattttatttattcttttaaaaataaagaggtggtgactaaacaatttcaaatctcatcacacatatggggtcagcccacaaaaataaagaacggtggaacggactgatatataatactaataaagaataggaaaaggaaagtgagtgaggtgcgagggagagaatttgtttaatatcagagtcgatcatgtgtcagttttatcgatatgattctgacttcaactgagtttaagcaattctgataaggcggagaaaatcatagtgctgagtctagaaaaatctcatgcagtgtgagataaacctcaaacaagaacatttgcggtgctaaacaatttcaagtcttatcacacatatatattatatattactaataaagaatagaaaaaggaaaggtaaacatcactaatgacagttgcggtgcaaagtgagtgagataataaacatcactaatagacatcactaacttttattggttatgtcaaactcaaaataaaatttctcaacttgtttacgtgcctatatataccatgcttgttatatgctcaaagcaccaaacaaaatttaaaaacactttgaacatttgcaaagaatggctgagaaagaagcaaatacccatgtcgtcctcttccccttgccaggccaagggcacatcggctcaatgttgaaactggcacagcttctttccaccgccggattctacgtcactttcgtccacaccgaacgcaactaccgtcgctacctcctcacctccacgtccttccacgtccccaagttccggttccgcaccatccccgacggttttcccgacgacgattcccgctcgcccctcccttttctcgagctccaagagtcgctggacacgaaatgtcgggggcattatcgggaattgttggtcgctgtcgacgaccaagaagagtggcccccagtcacttgtgtcgtggctgatcaagctcttccactctcactcgaagttcccgacgagttggggattcctgtaatgatactcgcaccacacagtgcgtgcagtatattgacgagttattcgattccggagcttataaggggaggtgaactccctatcccagatggggccaatatggatgaactattacaaggcgtactgggattggaaggtatcgtgaggcgtagggatatgtccatcagaagcgccaagtccatccaagatccatttcttcaattcgaagtgaaaatgagcaaaaacttgcccagaggaagagctctcatcctgaacactacagaatcgatagactctctttctttgcgacacattcggtcgatctgtcccactacctacgcactcgggcccttccacgtccttctcaggaacataaaagacgagtcccactccgcaagcctttccgaagaggacaggtcctgcatcgcctggctggactcgaaaccgaacaagtccgcggtctacgtgagtttcggtagcctcgccgccatggcgagagaagcatttcttgagtttcagcagggattgctcgacagcgggtattacttcttgtgggtgatccggcccgatatggtggaaggggggctggaagagagcgagctgaccgcgagcgaacaacgctactttgtgaagtgggccccacaggaggaggttcttgcgcacccggcggtagggtgtttcttgacgcacagcggttggaactctacgttggagagtatctttgcgggagtgccgatgatatgttggcctttctttgcggaccagctgattaacagtaggtttgcgagcgaggtgtggaaaattgccttggatatgaaggatttgtgcggaaggagccacgtggagaggatggtgaaggaagttatgagtggagagaaaggcgaagagctaaggaattctagctgcgagatggcagatagggtgaagaagagtgcagaggaaggtggctcttcctacgccaacttcaaagagttggttggacatatcaaatctttgagcttaccagcagaaagaggagaaaatggtggtgaaggaatgagtgtacaagcgccgagtaaacttttcctcctcaacgctgaggacggaaaacatgtccttaaaagtgacgaaccgtcggaacaaaggggtccacaatttaatccaaattttcttcggacctgagcttcggccatgctagagtccgcaaaaatcaccagtctctctctacaaatctatctctctctatttttctccagaataatgtgtgagtagttcccagataagggaattagggttcttatagggtttcgctcatgtgttgagcatataagaaacccttagtatgtatttgtatttgtaaaatacttctatcaataaaatttctaattcctaaaaccaaaatccagtgacctcgcttgagacgaagctttgacaggatatattggcgggtaaacctaagagaaaagagcgtttattagaataatcggatatttaaaagggcgtgaaaaggtttatccgttcgtccatttgtatgtgcatgccaaccacagggttcccctcgggatcaaagtactttgatccaacccctccgctgctatagtgcagtcggcttctgacgttcagtgcagccgtcatctgaaaacgacatgtcgcacaagtcctaagttacgcgacaggctgccgccctgcccttttcctggcgttttcttgtcgcgtgttttagtcgcataaagtagaatacttgcgactagaaccggagacattacgccatgaacaagagcgccgccgctggcctgctgggctatgcccgcgtcagcaccgacgaccaggacttgaccaaccaacgggccgaactgcacgcggccggctgcaccaagctgttttccgagaagatcaccggcaccaggcgcgaccgcccggagctggccaggatgcttgaccacctacgccctggcgacgttgtgacagtgaccaggctagaccgcctggcccgcagcacccgcgacctactggacattgccgagcgcatccaggaggccggcgcgggcctgcgtagcctggcagagccgtgggccgacaccaccacgccggccggccgcatggtgttgaccgtgttcgccggcattgccgagttcgagcgttccctaatcatcgaccgcacccggagcgggcgcgaggccgccaaggcccgaggcgtgaagtttggcccccgccctaccctcaccccggcacagatcgcgcacgcccgcgagctgatcgaccaggaaggccgcaccgtgaaagaggcggctgcactgcttggcgtgcatcgctcgaccctgtaccgcgcacttgagcgcagcgaggaagtgacgcccaccgaggccaggcggcgcggtgccttccgtgaggacgcattgaccgaggccgacgccctggcggccgccgagaatgaacgccaagaggaacaagcatgaaaccgcaccaggacggccaggacgaaccgtttttcattaccgaagagatcgaggcggagatgatcgcggccgggtacgtgttcgagccgcccgcgcacctctcaaccgtgcggctgcatgaaatcctggccggtttgtctgatgccaagctggcggcctggccggccagcttggccgctgaagaaaccgagcgccgccgtctaaaaaggtgatgtgtatttgagtaaaacagcttgcgtcatgcggtcgctgcgtatatgatccgatgagtaaataaacaaatacgcaaggggaacgcatgaaggttatcgctgtacttaaccagaaaggcgggtcaggcaagacgaccatcggaacccatctagcccgcgccctgcaactcgccggggccgatgttctgttagtcgattccgatccccagggcagtgcccgcgattgggcggccgtgcgggaagatcaaccgctaaccgttgtcggcatcgaccgcccgacgattgaccgcgacgtgaaggccatcggccggcgcgacttcgtagtgatcgacggagcgccccaggcggcggacttggctgtgtccgcgatcaaggcagccgacttcgtgctgattccggtgcagccaagcccttacgacatatgggccaccgccgacctggtggagctggttaagcagcgcattgaggtcacggatggaaggctacaagcggcctttgtcgtgtcgcgggcgatcaaaggcacgcgcatcggcggtgaggttgccgaggcgctggccgggtacgagctgcccattcttgagtcccgtatcacgcagcgcgtgagctacccaggcactgccgccgccggcacaaccgttcttgaatcagaacccgagggcgacgctgcccgcgaggtccaggcgctggccgctgaaattaaatcaaaactcatttgagttaatgaggtaaagagaaaatgagcaaaagcacaaacacgctaagtgccggccgtccgagcgcacgcagcagcaaggctgcaacgttggccagcctggcagacacgccagccatgaagcgggtcaactttcagttgccggcggaggatcacaccaagctgaagatgtacgcggtacgccaaggcaagaccattaccgagctgctatctgaatagatcgcgcagctaccagagtaaatgagcaaatgaataaatgagtagatgaattttagcggctaaaggaggcggcatggaaaatcaagaacaaccaggcaccgacgccgtggaatgccccatgtgtggaggaacgggcggttggccaggcgtaagcggctgggttgtctgccggccctgcaatggcactggaacccccaagcccgaggaatcggcgtgacggtcgcaaaccatccggcccggtacaaatcggcgcggcgctgggtgatgacctggtggagaagttgaaggccgcgcaggccgcccagcggcaacgcatcgaggcagaagcacgccccggtgaatcgtggcaagcggccgctgatcgaatccgcaaagaatcccggcaaccgccggcagccggtgcgccgtcgattaggaagccgcccaagggcgacgagcaaccagattttttcgttccgatgctctatgacgtgggcacccgcgatagtcgcagcatcatggacgtggccgttttccgtctgtcgaagcgtgaccgacgagctggcgaggtgatccgctacgagcttccagacgggcacgtagaggtttccgcagggccggccggcatggccagtgtgtgggattacgacctggtactgatggcggtttcccatctaaccgaatccatgaaccgataccgggaagggaagggagacaagcccggccgcgtgttccgtccacacgttgcggacgtactcaagttctgccggcgagccgatggcggaaagcagaaagacgacctggtagaaacctgcattcggttaaacaccacgcacgttgccatgcagcgtacgaagaaggccaagaacggccgcctggtgacggtatccgagggtgaagccttgattagccgctacaagatcgtaaagagcgaaaccgggcggccggagtacatcgagatcgagctagctgattggatgtaccgcgagatcacagaaggcaagaacccggacgtgctgacggttcaccccgattactttttgatcgatcccggcatcggccgttttctctaccgcctggcacgccgcgccgcaggcaaggcagaagccagatggttgttcaagacgatctacgaacgcagtggcagcgccggagagttcaagaagttctgtttcaccgtgcgcaagctgatcgggtcaaatgacctgccggagtacgatttgaaggaggaggcggggcaggctggcccgatcctagtcatgcgctaccgcaacctgatcgagggcgaagcatccgccggttcctaatgtacggagcagatgctagggcaaattgccctagcaggggaaaaaggtcgaaaaggactctttcctgtggatagcacgtacattgggaacccaaagccgtacattgggaaccggaacccgtacattgggaacccaaagccgtacattgggaaccggtcacacatgtaagtgactgatataaaagagaaaaaaggcgatttttccgcctaaaactctttaaaacttattaaaactcttaaaacccgcctggcctgtgcataactgtctggccagcgcacagccgaagagctgcaaaaagcgcctacccttcggtcgctgcgctccctacgccccgccgcttcgcgtcggcctatcgcggccgctggccgctcaaaaatggctggcctacggccaggcaatctaccagggcgcggacaagccgcgccgtcgccactcgaccgccggcgcccacatcaaggcaccctgcctcgcgcgtttcggtgatgacggtgaaaacctctgacacatgcagctcccggtgacggtcacagcttgtctgtaagcggatgccgggagcagacaagcccgtcagggcgcgtcagcgggtgttggcgggtgtcggggcgcagccatgacccagtcacgtagcgatagcggagtgtatactggcttaactatgcggcatcagagcagattgtactgagagtgcaccatatgcggtgtgaaataccgcacagatgcgtaaggagaaaataccgcatcaggcgctcttccgcttcctcgctcactgactcgctgcgctcggtcgttcggctgcggcgagcggtatcagctcactcaaaggcggtaatacggttatccacagaatcaggggataacgcaggaaagaacatgtgagcaaaaggccagcaaaaggccaggaaccgtaaaaaggccgcgttgctggcgtttttccataggctccgcccccctgacgagcatcacaaaaatcgacgctcaagtcagaggtggcgaaacccgacaggactataaagataccaggcgtttccccctggaagctccctcgtgcgctctcctgttccgaccctgccgcttaccggatacctgtccgcctttctcccttcgggaagcgtggcgctttctcatagctcacgctgtaggtatctcagttcggtgtaggtcgttcgctccaagctgggctgtgtgcacgaaccccccgttcagcccgaccgctgcgccttatccggtaactatcgtcttgagtccaacccggtaagacacgacttatcgccactggcagcagccactggtaacaggattagcagagcgaggtatgtaggcggtgctacagagttcttgaagtggtggcctaactacggctacactagaaggacagtatttggtatctgcgctctgctgaagccagttaccttcggaaaaagagttggtagctcttgatccggcaaacaaaccaccgctggtagcggtggtttttttgtttgcaagcagcagattacgcgcagaaaaaaaggatctcaagaagatcctttgatcttttctacggggtctgacgctcagtggaacgaaaactcacgttaagggattttggtcatgcattctaggtgattagaaaaactcatcgagcatcaaatgaaactgcaatttattcatatcaggattatcaataccatatttttgaaaaagccgtttctgtaatgaaggagaaaactcaccgaggcagttccataggatggcaagatcctggtatcggtctgcgattccgactcgtccaacatcaatacaacctattaatttcccctcgtcaaaaataaggttatcaagtgagaaatcaccatgagtgacgactgaatccggtgagaatggcaaaagtttatgcatttctttccagacttgttcaacaggccagccattacgctcgtcatcaaaatcactcgcatcaaccaaaccgttattcattcgtgattgcgcctgagcgagtcgaaatacgcgatcgctgttaaaaggacaattacaaacaggaatcgaatgcaaccggcgcaggaacactgccagcgcatcaacaatattttcacctgaatcaggatattcttctaatacctggaatgctgttttccctgggatcgcagtggtgagtaaccatgcatcatcaggagtacggataaaatgcttgatggtcggaagaggcataaattccgtcagccagtttagtctgaccatctcatctgtaacatcattggcaacgctacctttgccatgtttcagaaacaactctggcgcatcgggcttcccatacaatcggtagattgtcgcacctgattgcccgacattatcgcgagcccatttatacccatataaatcagcatccatgttggaatttaatcgcggccttgagcaagacgtttcccgttgaatatggctcataacagaacttattatttccttcctcttttctacagtatttaaagataccccaagaagctaattataacaagacgaactccaattcactgttccttgcattctaaaaccttaaataccagaaaacagctttttcaaagttgttttcaaagttggcgtataacatagtatcgacggagccgattttgaaaccgcggtgatcacaggcagcaacgctctgtcatcgttacaatcaacatgctaccctccgcgagatcatccgtgtttcaaacccggcagcttagttgccgttcttccgaatagcatcggtaacatgagcaaagtctgccgccttacaacggctctcccgctgacgccgtcccggactgatgggctgcctgtatcgagtggtgattttgtgccgagctgccggtcggggagctgttggctggctggtggcaggatatattgtggtgtaaacataacaagcttcgtctcagtca

SEQ ID NO: 35 - DNA, 43 bp, synthetic construct
  source 1..43: mol_type = other DNA; note = Forwrd primer pUPD2-Dom-pPAT-F
gcgccgtctcgctcgggagaatttgtcaaatcaggctcaaaga

SEQ ID NO: 36 - DNA, 45 bp, synthetic construct
  source 1..45: mol_type = other DNA; note = Reverse primer pUPD2-Dom-pPAT-R
gcgccgtctcgctcacattctttgcaaatgttcaaagtgttttta

SEQ ID NO: 37 - DNA, 20 bp, synthetic construct
  source 1..20: mol_type = other DNA; note = Actin-potato forward primer
gcttcccgatggtcaagtca

SEQ ID NO: 38 - DNA, 21 bp, synthetic construct
  source 1..21: mol_type = other DNA; note = Actin potato reverse primer
ggattccagctgcttccattc